European Patent Application EP 4 176 897 A1, published May 10, 2023. Title: Tuberculosis Compositions And Methods Of Using The Same. Applicant: International AIDS Vaccine Initiative, Inc. The sequence listing filed with the application follows.

SEQUENCE LISTING (98 sequences)

SEQ ID NO: 1 - DNA, 977 bp, synthetic construct
  source 1..977: mol_type = other DNA
  misc_feature 1..977: note = Description of Artificial Sequence: Mycobacterium Ag85B
atgacagacgtgagccgaaagattcgagcttggggacgccgattgatgatcggcacggcagcggctgtagtccttccgggcctggtggggcttgccgcggagcggcaaccgcgggcgcgttctcccggccggggctgccggtcgagtacctgcaggtgccgtcgccgtcgatgggccgcgacatcaaggttcagttccagagcggtgggaacaactcacctgcggtttatctgctcgacggcctgcgcgcccaagacgactacaacggctgggatatcaacaccccggcgttcgagtggtactaccagtcgggactgtcgatagtcatgccggtcggcgggcagtccagcttctacagcgactggtacagcccggcctgcggtaaggctggctgccagacttacaagtgggaaaccttcctgaccagcgagctgccgcaatggttgtccgccaacagggccgtgaagcccaccggcagcgctgcaatcggcttgtcgatggccggctcgtcggcaatgatcttggccgcctaccacccccagcagttcatctacgccggctcgctgtcggccctgctggacccctctcaggggatggggcctagcctgatcggcctcgcgatgggtgacgccggcggttacaaggccgcagacatgtggggtccctcgagtgacccggcatgggagcgcaacgaccctacgcagcagatccccaagctggtcgcaaacaacacccggctatgggtttattgcgggaacggcaccccgaacgagttgggcggtgccaacatacccgccgagttcttggagaacttcgttcgtagcagcaacctgaagttccaggatgcgtacaacgccgcgggcgggcacaacgccgtgttcaacttcccgcccaacggcacgcacagctgggagtactggggcgctcagctcaacgccatgaagggtgacctgcagagttcgttaggcgccggctga

SEQ ID NO: 2 - DNA, 858 bp, synthetic construct
  source 1..858: mol_type = other DNA
  misc_feature 1..858: note = Description of Artificial Sequence: Mycobacterium Ag85B (E. colioptimized)
atgtttagccgtcctggcctgccagttgaatacctgcaagttccgagcccgtccatgggtcgtgacattaaggtgcagttccagagcggcggtaacaatagcccggctgtgtacctgctggacggtctgcgtgcgcaggatgattacaacggctgggacatcaataccccggcatttgagtggtattaccagtcgggtctgagcattgtgatgccggttggcggtcaaagcagcttctatagcgattggtacagcccggcatgcggcaaggctggttgccaaacctacaagtgggaaactttcttgaccagcgagctgccgcaatggttgagcgccaaccgtgcggtcaaaccgaccggtagcgctgctattggcctgtccatggccggcagcagcgcgatgatcttggcggcataccatccgcagcagtttatctacgccggtagcctgagcgcattgctggacccgagccaaggcatgggtccgagcctgattggtctggcaatgggtgacgcaggtggttacaaagcggccgatatgtggggcccatctagcgacccggcatgggagcgtaatgacccgacccagcaaattccgaaactggtggcgaataacacgcgcctgtgggtctactgtggcaatggtacgccgaacgagctgggtggcgcgaatatccctgcggagtttctggaaaactttgttcgcagcagcaacctgaaattccaggacgcgtataacgcagccggtggtcacaatgcggttttcaatttcccgccaaatggcactcatagctgggagtactggggtgcgcagttgaacgcaatgaaaggcgatctgcaatcctctctgggtgcgggc

SEQ ID NO: 3 - DNA, 858 bp, synthetic construct
  source 1..858: mol_type = other DNA
  misc_feature 1..858: note = Description of Artificial Sequence: Mycobacterium Ag85B (humanoptimized)
atgttctccaggcccggcctgcctgtcgagtatctgcaggtcccctccccctccatgggcagagacatcaaggtgcagttccaatccggaggcaacaacagccccgccgtgtatctcctcgacggcctgagggctcaggacgactacaacggctgggacatcaacacccccgccttcgagtggtactaccagtccggactgagcatcgtcatgcccgtgggcggccagagctccttctacagcgactggtatagccctgcctgcggcaaagccggatgccagacctacaagtgggagacctttctgaccagcgaactgccccagtggctgtccgccaatagggccgtcaaacctaccggctccgctgccatcggactcagcatggccggaagctccgctatgatcctggccgcctaccacccccagcaatttatctacgctggcagcctgtccgctctgctggatcctagccaaggcatgggccctagcctcattggcctggccatgggcgatgctggcggctataaggccgccgatatgtggggccctagctccgatcctgcctgggagaggaatgaccccacccagcagatccccaagctggtggccaacaacacaaggctctgggtgtactgcggcaatggcacccccaacgaactgggcggagccaacattcccgccgagttcctggagaacttcgtcaggagcagcaacctgaagttccaggacgcctacaatgccgccggaggccacaacgctgtgttcaacttccctcccaacggcacccacagctgggagtattggggcgctcagctgaacgccatgaaaggcgacctccagagctccctgggagctgga

SEQ ID NO: 4 - protein, 325 aa, synthetic construct
  SOURCE 1..325
  REGION 1..325: NOTE = Description of Artificial Sequence: Mycobacterium Ag85B
MTDVSRKIRAWGRRLMIGTAAAVVLPGLVGLAGGAATAGAFSRPGLPVEYLQVPSPSMGRDIKVQFQSGGNNSPAVYLLDGLRAQDDYNGWDINTPAFEWYYQSGLSIVMPVGGQSSFYSDWYSPACGKAGCQTYKWETFLTSELPQWLSANRAVKPTGSAAIGLSMAGSSAMILAAYHPQQFIYAGSLSALLDPSQGMGPSLIGLAMGDAGGYKAADMWGPSSDPAWERNDPTQQIPKLVANNTRLWVYCGNGTPNELGGANIPAEFLENFVRSSNLKFQDAYNAAGGHNAVFNFPPNGTHSWEYWGAQLNAMKGDLQSSLGAG

SEQ ID NO: 5 - protein, 286 aa, synthetic construct
  SOURCE 1..286
  REGION 1..286: NOTE = Description of Artificial Sequence: Mycobacterium Ag85B (E. coliand human optimized)
MFSRPGLPVEYLQVPSPSMGRDIKVQFQSGGNNSPAVYLLDGLRAQDDYNGWDINTPAFEWYYQSGLSIVMPVGGQSSFYSDWYSPACGKAGCQTYKWETFLTSELPQWLSANRAVKPTGSAAIGLSMAGSSAMILAAYHPQQFIYAGSLSALLDPSQGMGPSLIGLAMGDAGGYKAADMWGPSSDPAWERNDPTQQIPKLVANNTRLWVYCGNGTPNELGGANIPAEFLENFVRSSNLKFQDAYNAAGGHNAVFNFPPNGTHSWEYWGAQLNAMKGDLQSSLGAG

SEQ ID NO: 6 - DNA, 288 bp, synthetic construct
  source 1..288: mol_type = other DNA
  misc_feature 1..288: note = Description of Artificial Sequence: Mycobacterium ESAT-6
atgacagagcagcagtggaatttcgcgggtatcgaggccgcggcaagcgcaatccagggaaatgtcacgtccattcattccctccttgacgaggggaagcagtccctgaccaagctcgcagcggcctggggcggtagcggttcggaggcgtaccagggtgtccagcaaaaatgggacgccacggctaccgagctgaacaacgcgctgcagaacctggcgcggacgatcagcgaagccggtcaggcaatggcttcgaccgaaggcaacgtcactgggatgttcgcatag

SEQ ID NO: 7 - DNA, 282 bp, synthetic construct
  source 1..282: mol_type = other DNA
  misc_feature 1..282: note = Description of Artificial Sequence: Mycobacterium ESAT-6 (humanoptimized)
accgagcagcagtggaacttcgccggcatcgaagctgccgctagcgccatccaaggcaacgtgaccagcatccacagcctgctggacgagggcaagcagagcctgaccaagctggctgctgcttggggcggatccggaagcgaagcctaccagggcgtgcagcagaagtgggacgccacagccaccgagctgaacaacgccctgcagaacctcgccagaaccatcagcgaggccggacaggctatggccagcacagagggcaatgtgaccggcatgttcgcc

SEQ ID NO: 8 - protein, 94 aa, synthetic construct
  SOURCE 1..94
  REGION 1..94: NOTE = Description of Artificial Sequence: ESAT-6
TEQQWNFAGIEAAASAIQGNVTSIHSLLDEGKQSLTKLAAAWGGSGSEAYQGVQQKWDATATELNNALQNLARTISEAGQAMASTEGNVTGMFA

SEQ ID NO: 9 - DNA, 687 bp, synthetic construct
  source 1..687: mol_type = other DNA
  misc_feature 1..687: note = Description of Artificial Sequence: Mycobacterium Rv1980c
gtgcgcatcaagatcttcatgctggtcacggctgtcgttttgctctgttgttcgggtgtggccacggccgcgcccaagacctactgcgaggagttgaaaggcaccgataccggccaggcgtgccagattcaaatgtccgacccggcctacaacatcaacatcagcctgcccagttactaccccgaccagaagtcgctggaaaattacatcgcccagacgcgcgacaagttcctcagcgcggccacatcgtccactccacgcgaagccccctacgaattgaatatcacctcggccacataccagtccgcgataccgccgcgtggtacgcaggccgtggtgctcaaggtctaccagaacgccggcggcacgcacccaacgaccacgtacaaggccttcgattgggaccaggcctatcgcaagccaatcacctatgacacgctgtggcaggctgacaccgatccgctgccagtcgtcttccccattgtgcaaggtgaactgagcaagcagaccggacaacaggtatcgatagcgccgaatgccggcttggacccggtgaattatcagaacttcgcagtcacgaacgacggggtgattttcttcttcaacccgggggagttgctgcccgaagcagccggcccaacccaggtattggtcccacgttccgcgatcgactcgatgctggcctag

SEQ ID NO: 10 - DNA, 690 bp, synthetic construct
  source 1..690: mol_type = other DNA
  misc_feature 1..690: note = Description of Artificial Sequence: Mycobacterium Rv1980c (humanoptimized)
atggtcaggatcaagatcttcatgctcgtgaccgccgtggtgctcctgtgttgttccggcgtggctaccgctgctcccaagacctactgcgaggagctgaagggaaccgacaccggccaggcctgccagatccaaatgagcgaccccgcctacaacatcaacatctccctcccctcctactaccccgatcagaagtccctcgagaactacatcgctcagaccagggacaagttcctgagcgccgccacaagcagcacacccagagaggccccctacgagctgaacatcacctccgccacctaccagtccgctattcctcccagaggcacccaggctgtggtgctcaaggtctaccaaaacgctggcggaacacaccccaccaccacctacaaggccttcgactgggaccaggcctacaggaagcccatcacatacgacaccctgtggcaggctgataccgatcccctgcccgtggtgttccccatcgtgcagggcgagctctccaagcagaccggccagcaagtgagcatcgcccccaatgctggactggaccccgtgaactaccagaacttcgccgtcaccaacgacggcgtgatcttcttcttcaatcccggcgaactgctgcctgaagctgctggccccacccaagtgctggtgcctagaagcgccatcgactccatgctggcctga

SEQ ID NO: 11 - protein, 228 aa, synthetic construct
  SOURCE 1..228
  REGION 1..228: NOTE = Description of Artificial Sequence: Rv1980c
VRIKIFMLVTAVVLLCCSGVATAAPKTYCEELKGTDTGQACQIQMSDPAYNINISLPSYYPDQKSLENYIAQTRDKFLSAATSSTPREAPYELNITSATYQSAIPPRGTQAVVLKVYQNAGGTHPTTTYKAFDWDQAYRKPITYDTLWQADTDPLPVVFPIVQGELSKQTGQQVSIAPNAGLDPVNYQNFAVTNDGVIFFFNPGELLPEAAGPTQVLVPRSAIDSMLA

SEQ ID NO: 12 - DNA, 1176 bp, synthetic construct
  source 1..1176: mol_type = other DNA
  misc_feature 1..1176: note = Description of Artificial Sequence: Mycobacterium Rv1039c
atggatttcggagctttaccccctgagatcaactccgcacgcatgtacgccggcgcgggtgcaggaccgatgatggccgccggggccgcatggaacggcctggccgccgagttgggtacgacggccgcgtcgtatgagtcggtgatcacccggctgaccaccgagtcgtggatgggtccggcctcgatggcgatggtcgccgcagcccagccctatctggcttggttgacctacaccgccgaagccgctgcgcatgccggctcgcaggccatggcgtcggcggccgcctacgaggcggcctatgcgatgacagtgccgccggaggtggtcgcggccaaccgggcgctgctggcggccctggtcgcgacgaacgtcctggggatcaacacaccggcaatcatggcgaccgaagccctctatgccgagatgtgggctcaggacgctctggctatgtacggctacgcggccgcttcgggagccgccgggatgctgcaaccgttaagcccgccgtcgcagaccaccaacccgggcgggctggccgcccagtccgccgcggtcggctcggctgccgccaccgccgccgtcaaccaggtgagcgtagcggacctgatcagtagcctgcccaacgcggtgagtgggctcgcctccccagtcacatcggttctcgactcgacggggctgagcggaatcattgccgacatcgacgccctgctcgcgaccccgttcgtggcaaacatcatcaacagcgcagtcaacaccgccgcttggtatgtcaacgccgccatccccaccgcgatattcctagcaaatgccctgaacagtggggcgccggtagcgatcgccgaaggcgccatcgaggctgccgagggtgccgccagtgcggccgccgcggggttggcggactcggtgacgccagcggggctcggcgcaagtttaggcgaggccaccctggtcggccggctgtcagtgccggcggcctggtctacggccgcaccggcgacaaccgccggcgccacagcgctcgaaggcagcggctggaccgtcgccgccgaagaagccggcccagttaccgggatgatgccgggaatggcctcggccgccaagggcaccggtgcctatgccgggccgcggtacggattcaagcccactgtcatgcccaaacaggtcgtcgtgtga

SEQ ID NO: 13 - DNA, 1176 bp, synthetic construct
  source 1..1176: mol_type = other DNA
  misc_feature 1..1176: note = Description of Artificial Sequence: Mycobacterium Rv1039c (humanoptimized)
atggattttggcgccctgcctcccgagatcaacagcgctaggatgtatgctggcgctggagccggacctatgatggccgctggagccgcctggaatggactggctgccgaactgggcacaacagccgcttcctacgagtccgtgatcaccagactcaccacagagtcctggatgggacctgccagcatggctatggtcgccgctgctcaaccctacctggcctggctgacctatacagctgaagccgctgctcacgccggaagccaagctatggctagcgccgccgcttatgaggccgcttatgccatgaccgtgcctcccgaggtcgtggctgccaacagagctctcctggccgccctcgtggctaccaacgtgctgggaatcaacacccccgctattatggccaccgaggctctgtacgctgagatgtgggcccaggatgccctcgccatgtacggatacgccgctgcttccggagctgctggaatgctgcagcccctgtcccccccttcccagaccaccaaccccggaggactggctgctcaaagcgctgctgtgggatccgctgctgctaccgctgccgtcaatcaggtcagcgtcgccgacctcatctccagcctgcctaacgctgtgagcggactggcctcccctgtcacatccgtgctcgatagcaccggcctgtccggcatcatcgccgacattgatgctctcctcgccaccccctttgtcgccaacatcatcaattccgccgtgaacaccgctgcctggtacgtcaacgctgccattcccaccgccatcttcctcgccaacgccctgaactccggagctcctgtcgccatcgctgagggcgctattgaggctgctgaaggagccgctagcgctgctgctgctggactggctgatagcgtcacccctgctggactcggagctagcctgggagaagccaccctggtcggcagactgtccgtgcctgctgcttggagcaccgctgctcctgctacaaccgctggagctaccgctctggagggatccggatggacagtggctgctgaggaagctggacccgtgaccggaatgatgcctggcatggccagcgctgctaagggaaccggcgcctatgccggacccagatacggattcaagcccaccgtcatgcccaagcaggtcgtcgtctaa

SEQ ID NO: 14 - protein, 391 aa, synthetic construct
  SOURCE 1..391
  REGION 1..391: NOTE = Description of Artificial Sequence: Rv1039c
MDFGALPPEINSARMYAGAGAGPMMAAGAAWNGLAAELGTTAASYESVITRLTTESWMGPASMAMVAAAQPYLAWLTYTAEAAAHAGSQAMASAAAYEAAYAMTVPPEVVAANRALLAALVATNVLGINTPAIMATEALYAEMWAQDALAMYGYAAASGAAGMLQPLSPPSQTTNPGGLAAQSAAVGSAAATAAVNQVSVADLISSLPNAVSGLASPVTSVLDSTGLSGIIADIDALLATPFVANIINSAVNTAAWYVNAAIPTAIFLANALNSGAPVAIAEGAIEAAEGAASAAAAGLADSVTPAGLGASLGEATLVGRLSVPAAWSTAAPATTAGATALEGSGWTVAAEEAGPVTGMMPGMASAAKGTGAYAGPRYGFKPTVMPKQVVV

SEQ ID NO: 15 - DNA, 1143 bp, synthetic construct
  source 1..1143: mol_type = other DNA
  misc_feature 1..1143: note = Description of Artificial Sequence: Mycobacterium Rv3136
atggatttcgcactgttaccaccggaagtcaactccgcccggatgtacaccggccctggggcaggatcgctgttggctgccgcgggcggctgggattcgctggccgccgagttggccaccacagccgaggcatatggatcggtgctgtccggactggccgccttgcattggcgtggaccggcagcggaatcgatggcggtgacggccgctccctatatcggttggctgtacacgaccgccgaaaagacacagcaaacagcgatccaagccagggcggcagcgctggccttcgagcaagcatacgcaatgaccctgccgccaccggtggtagcggccaaccggatacagctgctagcactgatcgcgacgaacttcttcggccagaacactgcggcgatcgcggccaccgaggcacagtacgccgagatgtgggcccaggacgccgccgcgatgtacggttacgccaccgcctcagcggctgcggccctgctgacaccgttctccccgccgcggcagaccaccaacccggccggcctgaccgctcaggccgccgcggtcagccaggccaccgacccactgtcgctgctgattgagacggtgacccaagcgctgcaagcgctgacgattccgagcttcatccctgaggacttcaccttccttgacgccatattcgctggatatgccacggtaggtgtgacgcaggatgtcgagtcctttgttgccgggaccatcggggccgagagcaacctaggccttttgaacgtcggcgacgagaatcccgcggaggtgacaccgggcgactttgggatcggcgagttggtttccgcgaccagtcccggcggtggggtgtctgcgtcgggtgccggcggtgcggcgagcgtcggcaacacggtgctcgcgagtgtcggccgggcaaactcgattgggcaactatcggtcccaccgagctgggccgcgccctcgacgcgccctgtctcggcattgtcgcccgccggcctgaccacactcccggggaccgacgtggccgagcacgggatgccaggtgtaccgggggtgccagtggcagcagggcgagcctccggcgtcctacctcgatacggggttcggctcacggtgatggcccacccacccgcggcagggtaa

SEQ ID NO: 16 - DNA, 1146 bp, synthetic construct
  source 1..1146: mol_type = other DNA
  misc_feature 1..1146: note = Description of Artificial Sequence: Mycobacterium Rv3136 (E. colioptimized)
atggattttgcgctgctgccgccggaagtgaacagcgcgcgcatgtataccggcccgggcgcgggcagcctgctggcggcggcgggcggctgggatagcctggcggcggaactggcgaccaccgcggaagcgtatggcagcgtgctgagcggcctggcggcgctgcattggcgcggcccggcggcggaaagcatggcggtgaccgcggcgccgtatattggctggctgtataccaccgcggaaaaaacccagcagaccgcgattcaggcgcgcgcggcggcgctggcgtttgaacaggcgtatgcgatgaccctgccgccgccggtggtggcggcgaaccgcattcagctgctggcgctgattgcgaccaacttttttggccagaacaccgcggcgattgcggcgaccgaagcgcagtatgcggaaatgtgggcgcaggatgcggcggcgatgtatggctatgcgaccgcgagcgcggcggcggcgctgctgaccccgtttagcccgccgcgccagaccaccaacccggcgggcctgaccgcgcaggcggcggcggtgagccaggcgaccgatccgctgagcctgctgattgaaaccgtgacccaggcgctgcaggcgctgaccattccgagctttattccggaagattttacctttctggatgcgatttttgcgggctatgcgaccgtgggcgtgacccaggatgtggaaagctttgtggcgggcaccattggcgcggaaagcaacctgggcctgctgaacgtgggcgatgaaaacccggcggaagtgaccccgggcgattttggcattggcgaactggtgagcgcgaccagcccgggcggcggcgtgagcgcgagcggcgcgggcggcgcggcgagcgtgggcaacaccgtgctggcgagcgtgggccgcgcgaacagcattggccagctgagcgtgccgccgagctgggcggcgccgagcacccgcccggtgagcgcgctgagcccggcgggcctgaccaccctgccgggcaccgatgtggcggaacatggcatgccgggcgtgccgggcgtgccggtggcggcgggccgcgcgagcggcgtgctgccgcgctatggcgtgcgcctgaccgtgatggcgcatccgccggcggcgggcgaattt

SEQ ID NO: 17 - DNA, 1143 bp, synthetic construct
  source 1..1143: mol_type = other DNA
  misc_feature 1..1143: note = Description of Artificial Sequence: Mycobacterium Rv3136 (humanoptimized)
atggatttcgctctgctcccccccgaggtgaatagcgctaggatgtacacaggacccggagctggaagcctcctggctgctgctggaggatgggactccctggctgccgagctcgctacaaccgctgaggcttacggaagcgtgctctccggcctggctgctctccattggagaggccctgctgccgagtccatggctgtcacagccgctccctacattggatggctgtacaccaccgccgagaagacccagcaaaccgctattcaggccagagctgccgccctggccttcgaacaggcctacgctatgacactccccccccctgtcgtggctgccaataggatccagctcctggccctcatcgccaccaacttcttcggccaaaacaccgctgccatcgctgccaccgaagcccagtacgccgaaatgtgggcccaggatgccgctgctatgtacggctatgccacagctagcgctgccgctgctctgctcacacccttcagcccccccaggcaaacaaccaaccctgccggactgacagcccaagctgctgccgtcagccaagctaccgaccccctgagcctcctgatcgaaaccgtgacacaggccctgcaggccctgaccattcccagctttatccccgaggacttcacctttctggacgctatcttcgctggctacgccaccgtgggcgtgacacaagacgtcgagtccttcgtcgccggcacaatcggagccgagtccaacctcggactcctcaacgtcggcgacgaaaatcccgccgaagtgacacctggagacttcggcattggagaactcgtcagcgccacatcccctggcggaggagtgagcgcttccggagctggaggagctgcttccgtgggcaataccgtgctggccagcgtgggaagggccaactccattggccagctcagcgtccccccttcctgggctgccccttccacaaggcctgtgtccgctctcagccctgctggactgaccacactccctggcacagacgtggctgagcatggcatgcccggagtgcctggagtccctgtggctgctggcagagcttccggagtcctccctaggtatggcgtgaggctgacagtgatggctcatccccccgctgccggataa

SEQ ID NO: 18 - protein, 380 aa, synthetic construct
  SOURCE 1..380
  REGION 1..380: NOTE = Description of Artificial Sequence: Rv3136
MDFALLPPEVNSARMYTGPGAGSLLAAAGGWDSLAAELATTAEAYGSVLSGLAALHWRGPAAESMAVTAAPYIGWLYTTAEKTQQTAIQARAAALAFEQAYAMTLPPPVVAANRIQLLALIATNFFGQNTAAIAATEAQYAEMWAQDAAAMYGYATASAAAALLTPFSPPRQTTNPAGLTAQAAAVSQATDPLSLLIETVTQALQALTIPSFIPEDFTFLDAIFAGYATVGVTQDVESFVAGTIGAESNLGLLNVGDENPAEVTPGDFGIGELVSATSPGGGVSASGAGGAASVGNTVLASVGRANSIGQLSVPPSWAAPSTRPVSALSPAGLTTLPGTDVAEHGMPGVPGVPVAAGRASGVLPRYGVRLTVMAHPPAAG

SEQ ID NO: 19 - DNA, 312 bp, synthetic construct
  source 1..312: mol_type = other DNA
  misc_feature 1..312: note = Description of Artificial Sequence: Mycobacterium Rv3615c
atgacggaaaacttgaccgtccagcccgagcgtctcggtgtactggcgtcgcaccatgacaacgcggcggtcgatgcctcctcgggcgtcgaagctgccgctggcctaggcgaatctgtggcgatcactcacggtccgtactgctcacagttcaacgacacgttaaatgtgtacttgactgcccacaatgccctgggctcgtccttgcatacggccggtgtcgatctcgccaaaagtcttcgaattgcggcgaagatatatagcgaggccgacgaagcgtggcgcaaggctatcgacgggttgtttacctga

SEQ ID NO: 20 - DNA, 312 bp, synthetic construct
  source 1..312: mol_type = other DNA
  misc_feature 1..312: note = Description of Artificial Sequence: Mycobacterium Rv3615c (humanoptimized)
atgaccgagaacctgaccgtgcagcctgagaggctgggagtgctggccagccaccacgacaacgctgccgtggacgcttccagcggagtggaggctgctgctggactgggagagagcgtggccatcacccacggaccctactgcagccagttcaacgacaccctgaacgtgtacctgacagcccacaacgccctgggaagcagcctgcatacagccggcgtggacctggctaagtccctgaggatcgccgccaagatctacagcgaggccgacgaggcctggaggaaagccatcgacggcctgttcacctaa

SEQ ID NO: 21 - protein, 103 aa, synthetic construct
  SOURCE 1..103
  REGION 1..103: NOTE = Description of Artificial Sequence: Rv3615c
MTENLTVQPERLGVLASHHDNAAVDASSGVEAAAGLGESVAITHGPYCSQFNDTLNVYLTAHNALGSSLHTAGVDLAKSLRIAAKIYSEADEAWRKAIDGLFT

SEQ ID NO: 22 - DNA, 633 bp, synthetic construct
  source 1..633: mol_type = other DNA
  misc_feature 1..633: note = Description of Artificial Sequence: Mycobacterium Rv1733c
atgatcgccacaacccgcgatcgtgaaggagccaccatgatcacgtttaggctgcgcttgccgtgccggacgatactgcgggtgttcagccgcaatccgctggtgcgtgggacggatcgactcgaggcggtcgtcatgctgctggccgtcacggtctcgctgctgactatcccgttcgccgccgcggccggcaccgcagtccaggattcccgcagccacgtctatgcccaccaggcccagacccgccatcccgcaaccgcgaccgtgatcgatcacgagggggtgatcgacagcaacacgaccgccacgtcagcgccgccgcgcacgaagatcaccgtgcctgcccgatgggtcgtgaacggaatagaacgcagcggtgaggtcaacgcgaagccgggaaccaaatccggtgaccgcgtcggcatttgggtcgacagtgccggtcagctggtcgatgaaccagctccgccggcccgtgccattgcggatgcggccctggccgccttgggactctggttgagcgtcgccgcggttgcgggcgccctgctggcgctcactcgggcgattctgatccgcgttcgcaacgccagttggcaacacgacatcgacagcctgttctgcacgcagcggtga

SEQ ID NO: 23 - DNA, 630 bp, synthetic construct
  source 1..630: mol_type = other DNA
  misc_feature 1..630: note = Description of Artificial Sequence: Mycobacterium Rv1733c (E. colioptimized)
atgattgcgactacccgtgatcgtgagggcgcgaccatgatcacgttccgtctgcgtctgccgtgtcgcaccattttgcgcgtgttttcgcgtaacccgctggtccgcggtaccgaccgtctggaggccgttgtcatgctgctggcggttaccgtgagcctgctgacgatcccattcgcagcggcagctggcacggccgtccaagacagccgtagccatgtgtatgctcaccaggctcaaacccgtcacccggctactgccactgttatcgatcacgaaggcgtgattgactccaataccacggcaacctccgcaccgcctcgcaccaagattacggttcctgcgcgttgggtggtgaatggtattgaacgcagcggcgaagttaatgccaaaccgggtaccaaaagcggtgaccgtgtgggcatctgggtcgatagcgccggtcagctggtcgacgagccggcaccgccagcgcgtgcgatcgccgatgcggcgctggctgccctgggtctgtggctgagcgtggcagcggtcgccggtgcgttgctggcgctgacgcgcgcaattctgatccgcgttcgcaatgcgagctggcagcacgatattgatagcctgttttgcacccaacgt

SEQ ID NO: 24 - protein, 210 aa, synthetic construct
  SOURCE 1..210
  REGION 1..210: NOTE = Description of Artificial Sequence: Rv1733c
MIATTRDREGATMITFRLRLPCRTILRVFSRNPLVRGTDRLEAVVMLLAVTVSLLTIPFAAAAGTAVQDSRSHVYAHQAQTRHPATATVIDHEGVIDSNTTATSAPPRTKITVPARWVVNGIERSGEVNAKPGTKSGDRVGIWVDSAGQLVDEPAPPARAIADAALAALGLWLSVAAVAGALLALTRAILIRVRNASWQHDIDSLFCTQR

SEQ ID NO: 25 - DNA, 504 bp, synthetic construct
  source 1..504: mol_type = other DNA
  misc_feature 1..504: note = Description of Artificial Sequence: Mycobacterium Rv1733c(transmembrane deleted; E. coli optimized)
atgattgcgactacccgtgatcgtgagggcgcgaccatgatcacgttccgtctgcgtctgccgtgtcgcaccattttgcgcgtgttttcgcgtaacccgctggtccgcggtaccgaccgtctggaggcccccggggtccaagacagccgtagccatgtgtatgctcaccaggctcaaacccgtcacccggctactgccactgttatcgatcacgaaggcgtgattgactccaataccacggcaacctccgcaccgcctcgcaccaagattacggttcctgcgcgttgggtggtgaatggtattgaacgcagcggcgaagttaatgccaaaccgggtaccaaaagcggtgaccgtgtgggcatctgggtcgatagcgccggtcagctggtcgacgagccggcaccgccagcgcgtgcgatcgccgattctagacgcgcaattctgatccgcgttcgcaatgcgagctggcagcacgatattgatagcctgttttgcacccaacgt

SEQ ID NO: 26 - DNA, 489 bp, synthetic construct
  source 1..489: mol_type = other DNA
  misc_feature 1..489: note = Description of Artificial Sequence: Mycobacterium Rv1733c(transmembrane deleted; human optimized)
atcgccaccaccagggacagggaaggcgctaccatgatcaccttcaggctgaggctcccctgcaggaccatcctgagggtgttcagcaggaaccccctggtgaggggcaccgacagactggaagccgtgcaggacagcaggagccacgtgtatgcccaccaggctcagaccaggcaccctgctaccgccaccgtgatcgaccacgagggcgtgatcgactccaacaccaccgccaccagcgctcctcccagaaccaagatcacagtgcccgccaggtgggtggtgaacggcatcgagaggagcggcgaggtgaacgccaagcctggaaccaagagcggcgacagggtgggcatttgggtcgatagcgccggccagctggtggatgaacctgctccccctgccagagccatcgccgatagggccatcctgatcagggtgaggaacgccagctggcagcacgacatcgacagcctgttctgcacccaaagg

SEQ ID NO: 27 - protein, 168 aa, synthetic construct
  SOURCE 1..168
  REGION 1..168: NOTE = Description of Artificial Sequence: Rv1733c (both transmembraneregions deleted; E. coli optimized)
MIATTRDREGATMITFRLRLPCRTILRVFSRNPLVRGTDRLEAPGVQDSRSHVYAHQAQTRHPATATVIDHEGVIDSNTTATSAPPRTKITVPARWVVNGIERSGEVNAKPGTKSGDRVGIWVDSAGQLVDEPAPPARAIADSRRAILIRVRNASWQHDIDSLFCTQR

SEQ ID NO: 28 - protein, 163 aa, synthetic construct
  SOURCE 1..163
  REGION 1..163: NOTE = Description of Artificial Sequence: Rv1733c (both transmembraneregions deleted; human optimized)
IATTRDREGATMITFRLRLPCRTILRVFSRNPLVRGTDRLEAVQDSRSHVYAHQAQTRHPATATVIDHEGVIDSNTTATSAPPRTKITVPARWVVNGIERSGEVNAKPGTKSGDRVGIWVDSAGQLVDEPAPPARAIADRAILIRVRNASWQHDIDSLFCTQR

SEQ ID NO: 29 - DNA, 432 bp, synthetic construct
  source 1..432: mol_type = other DNA
  misc_feature 1..432: note = Description of Artificial Sequence: Mycobacterium Rv2626c
atgaccaccgcacgcgacatcatgaacgcaggtgtgacctgtgttggcgaacacgagacgctaaccgctgccgctcaatacatgcgtgagcacgacatcggcgcgttgccgatctgcggggacgacgaccggctgcacggcatgctcaccgaccgcgacattgtgatcaaaggcctggctgcgggcctagacccgaataccgccacggctggcgagttggcccgggacagcatctactacgtcgatgcgaacgcaagcatccaggagatgctcaacgtcatggaagaacatcaggtccgccgtgttccggtcatctcagagcaccgcttggtcggaatcgtcaccgaagccgacatcgcccgacacctgcccgagcacgccattgtgcagttcgtcaaggcaatctgctcgcccatggccctcgccagctag

SEQ ID NO: 30 - DNA, 428 bp, synthetic construct
  source 1..428: mol_type = other DNA
  misc_feature 1..428: note = Description of Artificial Sequence: Mycobacterium Rv2626c (E. colioptimized)
atgaccacggcgcgtgatatcatgaatgcgggtgtcacctgtgttggcgagcacgaaacgttgaccgcagcagcacagtacatgcgcgaacatgatatcggcgcattgccgatttgcggcgacgatgatcgtctgcacggtatgctgaccgaccgcgatatcgttatcaagggtctggccgcaggcttggacccgaacaccgcgaccgccggtgaactggcacgtgacagcatctattacgtcgacgcgaacgccagcattcaagagatgctgaacgtgatggaagagcatcaggtgcgtcgtgtcccggttatcagcgaacatcgtctggttggtatcgttaccgaagccgacatcgcacgtcacctgccggagcacgcgattgttcagttcgtgaaagcgatttgcagcccgatggcgttggcgtc

SEQ ID NO: 31 - DNA, 426 bp, synthetic construct
  source 1..426: mol_type = other DNA
  misc_feature 1..426: note = Description of Artificial Sequence: Mycobacterium Rv2626c (humanoptimized)
acaacagccagggacatcatgaacgccggcgtgacctgcgtgggagagcatgaaaccctcaccgccgccgcccaatacatgagggagcacgacatcggcgccctgcccatctgtggagacgacgacaggctgcacggcatgctgaccgacagggacatcgtgatcaagggcctggctgccggcctcgatcctaacaccgctacagccggcgagctggccagagacagcatctactacgtggacgccaacgccagcatccaggagatgctcaacgtgatggaggagcaccaggtgagaagggtgcctgtgatcagcgagcacaggctggtgggcatcgtgaccgaggccgatatcgctaggcacctgcccgagcacgccatcgtgcagttcgtgaaggccatctgcagccccatggctctggccagc

SEQ ID NO: 32 - protein, 143 aa, synthetic construct
  SOURCE 1..143
  REGION 1..143: NOTE = Description of Artificial Sequence: Rv2626c
MTTARDIMNAGVTCVGEHETLTAAAQYMREHDIGALPICGDDDRLHGMLTDRDIVIKGLAAGLDPNTATAGELARDSIYYVDANASIQEMLNVMEEHQVRRVPVISEHRLVGIVTEADIARHLPEHAIVQFVKAICSPMALAS

SEQ ID NO: 33 - DNA, 300 bp, synthetic construct
  source 1..300: mol_type = other DNA
  misc_feature 1..300: note = Description of Artificial Sequence: Mycobacterium Rv3407
atgcgtgctaccgttgggcttgtggaggcaatcggaatccgagaactaagacagcacgcatcgcgatacctcgcccgggttgaagccggcgaggaacttggcgtcaccaacaaaggaagacttgtggcccgactcatcccggtgcaggccgcggagcgttctcgcgaagccctgattgaatcaggtgtcctgattccggctcgtcgtccacaaaaccttctcgacgtcaccgccgaaccggcgcgcggccgcaagcgcaccctgtccgatgttctcaacgaaatgcgcgacgagcagtga

SEQ ID NO: 34 - DNA, 297 bp, synthetic construct
  source 1..297: mol_type = other DNA
  misc_feature 1..297: note = Description of Artificial Sequence: Mycobacterium Rv3407 (E. colioptimized)
atgcgtgcgactgtgggtctggttgaggcgattggcattcgcgagctgcgccaacatgccagccgttacttggctcgtgtcgaggcgggtgaagaactgggcgtgacgaataagggtcgtctggtcgcccgtctgattccggttcaggcagctgagcgttctcgcgaggcgctgattgaatccggcgtcctgatcccggctcgccgtccgcaaaacctgctggacgtgacggcggagccagctcgtggtcgcaaacgcacgctgtctgatgtcctgaacgaaatgcgcgacgagcag

SEQ ID NO: 35 - DNA, 297 bp, synthetic construct
  source 1..297: mol_type = other DNA
  misc_feature 1..297: note = Description of Artificial Sequence: Mycobacterium Rv3407 (humanoptimized)
atgagggcgaccgtcgggctggtggaggcgataggtatccgggagttgcgacagcacgcatcacgatatctggcacgggtggaagctggggaggaactgggcgtgaccaacaaggggcggctggtcgcgaggctgatccccgtgcaggccgccgagcggtcccgcgaagccctcatcgagtctggggtgctcattccagcacgcaggccgcaaaatctcctggacgtcactgcggagcccgccagaggcagaaagaggacgctgagtgacgtgctgaacgagatgagggacgaacag

SEQ ID NO: 36 - protein, 99 aa, synthetic construct
  SOURCE 1..99
  REGION 1..99: NOTE = Description of Artificial Sequence: Rv3407
MRATVGLVEAIGIRELRQHASRYLARVEAGEELGVTNKGRLVARLIPVQAAERSREALIESGVLIPARRPQNLLDVTAEPARGRKRTLSDVLNEMRDEQ

SEQ ID NO: 37 - DNA, 363 bp, synthetic construct
  source 1..363: mol_type = other DNA
  misc_feature 1..363: note = Description of Artificial Sequence: Mycobacterium Rv2628c
atgtccacgcaacgaccgaggcactccggtattcgggctgttggcccctacgcatgggccggccgatgtggtcggataggcaggtggggggtgcaccaggaggcgatgatgaatctagcgatatggcacccgcgcaaggtgcaatccgccaccatctatcaggtgaccgatcgctcgcacgacgggcgcacagcacgggtgcctggtgacgagatcactagcaccgtgtccggttggttgtcggagttgggcacccaaagcccgttggccgatgagcttgcgcgtgcggtgcggatcggcgactggcccgctgcgtacgcaatcggtgagcacctgtccgttgagattgccgttgcggtctaa

SEQ ID NO: 38 - DNA, 363 bp, synthetic construct
  source 1..363: mol_type = other DNA
  misc_feature 1..363: note = Description of Artificial Sequence: Mycobacterium Rv2628c (humanoptimized)
atgagcacccagagacccaggcacagcggcattagggccgtgggaccttatgcttgggccggcagatgcggaaggatcggcagatggggcgtgcaccaagaggccatgatgaacctggccatctggcaccccaggaaggtgcagagcgccaccatctaccaggtgaccgacaggagccatgacggaaggaccgccagagtgcccggcgatgagatcaccagcaccgtgagcggctggctgagcgaactgggcacccaatcccccctggctgatgaactggccagggctgtgaggatcggcgattggcctgccgcctatgccatcggcgagcatctgagcgtggagatcgccgtggccgtgtaa

SEQ ID NO: 39 - protein, 120 aa, synthetic construct
  SOURCE 1..120
  REGION 1..120: NOTE = Description of Artificial Sequence: Rv2628c
MSTQRPRHSGIRAVGPYAWAGRCGRIGRWGVHQEAMMNLAIWHPRKVQSATIYQVTDRSHDGRTARVPGDEITSTVSGWLSELGTQSPLADELARAVRIGDWPAAYAIGEHLSVEIAVAV

SEQ ID NO: 40 - DNA, 1089 bp, synthetic construct
  source 1..1089: mol_type = other DNA
  misc_feature 1..1089: note = Description of Artificial Sequence: Mycobacterium Rv1009
atgttgcgcctggtagtcggtgcgctgctgctggtgttggcgttcgccggtggctatgcggtcgccgcatgcaaaacggtgacgttgaccgtcgacggaaccgcgatgcgggtgaccacgatgaaatcgcgggtgatcgacatcgtcgaagagaacgggttctcagtcgacgaccgcgacgacctgtatcccgcggccggcgtgcaggtccatgacgccgacaccatcgtgctgcggcgtagccgtccgctgcagatctcgctggatggtcacgacgctaagcaggtgtggacgaccgcgtcgacggtggacgaggcgctggcccaactcgcgatgaccgacacggcgccggccgcggcttctcgcgccagccgcgtcccgctgtccgggatggcgctaccggtcgtcagcgccaagacggtgcagctcaacgacggcgggttggtgcgcacggtgcacttgccggcccccaatgtcgcggggctgctgagtgcggccggcgtgccgctgttgcaaagcgaccacgtggtgcccgccgcgacggccccgatcgtcgaaggcatgcagatccaggtgacccgcaatcggatcaagaaggtcaccgagcggctgccgctgccgccgaacgcgcgtcgtgtcgaggacccggagatgaacatgagccgggaggtcgtcgaagacccgggggttccggggacccaggatgtgacgttcgcggtagctgaggtcaacggcgtcgagaccggccgtttgcccgtcgccaacgtcgtggtgaccccggcccacgaagccgtggtgcgggtgggcaccaagcccggtaccgaggtgcccccggtgatcgacggaagcatctgggacgcgatcgccggctgtgaggccggtggcaactgggcgatcaacaccggcaacgggtattacggtggtgtgcagtttgaccagggcacctgggaggccaacggcgggctgcggtatgcaccccgcgctgacctcgccacccgcgaagagcagatcgccgttgccgaggtgacccgactgcgtcaaggttggggcgcctggccggtatgtgctgcacgagcgggtgcgcgctga

SEQ ID NO: 41 - DNA, 1023 bp, synthetic construct
  source 1..1023: mol_type = other DNA
  misc_feature 1..1023: note = Description of Artificial Sequence: Mycobacterium Rv1009 (signalsequence deleted)
gcatgcaaaacggtgacgttgaccgtcgacggaaccgcgatgcgggtgaccacgatgaaatcgcgggtgatcgacatcgtcgaagagaacgggttctcagtcgacgaccgcgacgacctgtatcccgcggccggcgtgcaggtccatgacgccgacaccatcgtgctgcggcgtagccgtccgctgcagatctcgctggatggtcacgacgctaagcaggtgtggacgaccgcgtcgacggtggacgaggcgctggcccaactcgcgatgaccgacacggcgccggccgcggcttctcgcgccagccgcgtcccgctgtccgggatggcgctaccggtcgtcagcgccaagacggtgcagctcaacgacggcgggttggtgcgcacggtgcacttgccggcccccaatgtcgcggggctgctgagtgcggccggcgtgccgctgttgcaaagcgaccacgtggtgcccgccgcgacggccccgatcgtcgaaggcatgcagatccaggtgacccgcaatcggatcaagaaggtcaccgagcggctgccgctgccgccgaacgcgcgtcgtgtcgaggacccggagatgaacatgagccgggaggtcgtcgaagacccgggggttccggggacccaggatgtgacgttcgcggtagctgaggtcaacggcgtcgagaccggccgtttgcccgtcgccaacgtcgtggtgaccccggcccacgaagccgtggtgcgggtgggcaccaagcccggtaccgaggtgcccccggtgatcgacggaagcatctgggacgcgatcgccggctgtgaggccggtggcaactgggcgatcaacaccggcaacgggtattacggtggtgtgcagtttgaccagggcacctgggaggccaacggcgggctgcggtatgcaccccgcgctgacctcgccacccgcgaagagcagatcgccgttgccgaggtgacccgactgcgtcaaggttggggcgcctggccggtatgtgctgcacgagcgggtgcgcgctga

SEQ ID NO: 42 - protein, 362 aa, synthetic construct
  SOURCE 1..362
  REGION 1..362: NOTE = Description of Artificial Sequence: RpfB (mycobacterial sequence)
MLRLVVGALLLVLAFAGGYAVAACKTVTLTVDGTAMRVTTMKSRVIDIVEENGFSVDDRDDLYPAAGVQVHDADTIVLRRSRPLQISLDGHDAKQVWTTASTVDEALAQLAMTDTAPAAASRASRVPLSGMALPVVSAKTVQLNDGGLVRTVHLPAPNVAGLLSAAGVPLLQSDHVVPAATAPIVEGMQIQVTRNRIKKVTERLPLPPNARRVEDPEMNMSREVVEDPGVPGTQDVTFAVAEVNGVETGRLPVANVVVTPAHEAVVRVGTKPGTEVPPVIDGSIWDAIAGCEAGGNWAINTGNGYYGGVQFDQGTWEANGGLRYAPRADLATREEQIAVAEVTRLRQGWGAWPVCAARAGAR

SEQ ID NO: 43 - protein, 340 aa, synthetic construct
  SOURCE 1..340
  REGION 1..340: NOTE = Description of Artificial Sequence: RpfB (mycobacterial sequence;signal sequence deleted)
ACKTVTLTVDGTAMRVTTMKSRVIDIVEENGFSVDDRDDLYPAAGVQVHDADTIVLRRSRPLQISLDGHDAKQVWTTASTVDEALAQLAMTDTAPAAASRASRVPLSGMALPVVSAKTVQLNDGGLVRTVHLPAPNVAGLLSAAGVPLLQSDHVVPAATAPIVEGMQIQVTRNRIKKVTERLPLPPNARRVEDPEMNMSREVVEDPGVPGTQDVTFAVAEVNGVETGRLPVANVVVTPAHEAVVRVGTKPGTEVPPVIDGSIWDAIAGCEAGGNWAINTGNGYYGGVQFDQGTWEANGGLRYAPRADLATREEQIAVAEVTRLRQGWGAWPVCAARAGAR

SEQ ID NO: 44 - DNA, 465 bp, synthetic construct
  source 1..465: mol_type = other DNA
  misc_feature 1..465: note = Description of Artificial Sequence: Mycobacterium Rv2389c
atgacaccgggtttgcttactactgcgggtgctggccgaccacgtgacaggtgcgccaggatcgtatgcacggtgttcatcgaaaccgccgttgtcgcgaccatgtttgtcgcgttgttgggtctgtccaccatcagctcgaaagccgacgacatcgattgggacgccatcgcgcaatgcgaatccggcggcaattgggcggccaacaccggtaacgggttatacggtggtctgcagatcagccaggcgacgtgggattccaacggtggtgtcgggtcgccggcggccgcgagtccccagcaacagatcgaggtcgcagacaacattatgaaaacccaaggcccgggtgcgtggccgaaatgtagttcttgtagtcagggagacgcaccgctgggctcgctcacccacatcctgacgttcctcgcggccgagactggaggttgttcggggagcagggacgattga

SEQ ID NO: 45 - DNA, 354 bp, synthetic construct
  source 1..354: mol_type = other DNA
  misc_feature 1..354: note = Description of Artificial Sequence: Mycobacterium Rv2389c (E. colioptimized; leader sequence deleted)
aagcttttgctgggcctgagcaccattagcagcaaagcggatgacatcgactgggatgcgattgcgcagtgtgagagcggtggcaattgggcagcgaataccggcaatggcctgtacggcggtctgcagatctcccaggcgacgtgggacagcaatggtggcgtcggcagcccggctgccgcgtccccacaacaacagatcgaggtggcagataacattatgaaaacgcagggtccgggtgcttggccaaaatgctccagctgcagccagggtgacgcaccgctgggcagcctgacccacattctgacgttcctggcagcggaaaccggtggttgtagcggtagccgcgatgac

SEQ ID NO: 46 - DNA, 465 bp, synthetic construct
  source 1..465: mol_type = other DNA
  misc_feature 1..465: note = Description of Artificial Sequence: Mycobacterium Rv2389c (humanoptimized; leader sequence present)
acccccggactcctcaccacagctggagctggcaggcccagagacagatgcgccaggatcgtgtgcaccgtgttcatcgagaccgccgtggtggctaccatgttcgtggccctgctgggcctgagcaccatcagcagcaaggccgacgacatcgactgggacgccatcgcccagtgtgaatccggcggaaactgggccgccaataccggcaatggcctgtacggcggcctgcagatcagccaggctacctgggactccaacggaggagtgggaagccctgccgctgcttcccctcagcagcagatcgaggtggccgacaacatcatgaagacccaaggccctggcgcctggcctaagtgttccagctgtagccagggcgatgctcctctgggcagcctgacccacatcctgacctttctcgccgccgagacaggcggatgtagcggaagcagggacgactaatga

SEQ ID NO: 47 - protein, 116 aa, synthetic construct
  SOURCE 1..116
  REGION 1..116: NOTE = Description of Artificial Sequence: RpfD (E. coli optimized)
LLGLSTISSKADDIDWDAIAQCESGGNWAANTGNGLYGGLQISQATWDSNGGVGSPAAASPQQQIEVADNIMKTQGPGAWPKCSSCSQGDAPLGSLTHILTFLAAETGGCSGSRDD

SEQ ID NO: 48 - protein, 153 aa, synthetic construct
  SOURCE 1..153
  REGION 1..153: NOTE = Description of Artificial Sequence: RpfD (mycobacterial sequenceand human optimized)
TPGLLTTAGAGRPRDRCARIVCTVFIETAVVATMFVALLGLSTISSKADDIDWDAIAQCESGGNWAANTGNGLYGGLQISQATWDSNGGVGSPAAASPQQQIEVADNIMKTQGPGAWPKCSSCSQGDAPLGSLTHILTFLAAETGGCSGSRDD

SEQ ID NO: 49 - DNA, 519 bp, synthetic construct
  source 1..519: mol_type = other DNA
  misc_feature 1..519: note = Description of Artificial Sequence: Mycobacterium Rv2450c
ttgaagaacgcccgtacgacgctcatcgccgccgcgattgccgggacgttggtgaccacgtcaccagccggtatcgccaatgccgacgacgcgggcttggacccaaacgccgcagccggcccggatgccgtgggctttgacccgaacctgccgccggccccggacgctgcacccgtcgatactccgccggctccggaggacgcgggctttgatcccaacctccccccgccgctggccccggacttcctgtccccgcctgcggaggaagcgcctcccgtgcccgtggcctacagcgtgaactgggacgcgatcgcgcagtgcgagtccggtggaaactggtcgatcaacaccggtaacggttactacggcggcctgcggttcaccgccggcacctggcgtgccaacggtggctcggggtccgcggccaacgcgagccgggaggagcagatccgggtggctgagaacgtgctgcgttcgcagggtatccgcgcctggccggtctgcggccgccgcggctga

SEQ ID NO: 50 - protein, 172 aa, synthetic construct
  SOURCE 1..172
  REGION 1..172: NOTE = Description of Artificial Sequence: RpfE
LKNARTTLIAAAIAGTLVTTSPAGIANADDAGLDPNAAAGPDAVGFDPNLPPAPDAAPVDTPPAPEDAGFDPNLPPPLAPDFLSPPAEEAPPVPVAYSVNWDAIAQCESGGNWSINTGNGYYGGLRFTAGTWRANGGSGSAANASREEQIRVAENVLRSQGIRAWPVCGRRG

SEQ ID NO: 51 - DNA, 1584 bp, synthetic construct
  source 1..1584: mol_type = other DNA
  misc_feature 1..1584: note = Description of Artificial Sequence: Mycobacterium ESAT6-Rv1733c-Rv2626c-RpfD fusion protein (E. coli optimized)
atgacagagcagcagtggaatttcgcgggtatcgaggccgcggcaagcgcaatccagggaaatgtcacgtccattcattccctccttgacgaggggaagcagtccctgaccaagctcgcagcggcctggggcggtagcggttcggaggcgtaccagggtgtccagcaaaaatgggacgccacggctaccgagctgaacaacgcgctgcagaacctggcgcggacgatcagcgaagccggtcaggcaatggcttcgaccgaaggcaacgtcactgggatgttcgcagaattcatgattgcgactacccgtgatcgtgagggcgcgaccatgatcacgttccgtctgcgtctgccgtgtcgcaccattttgcgcgtgttttcgcgtaacccgctggtccgcggtaccgaccgtctggaggcccccggggtccaagacagccgtagccatgtgtatgctcaccaggctcaaacccgtcacccggctactgccactgttatcgatcacgaaggcgtgattgactccaataccacggcaacctccgcaccgcctcgcaccaagattacggttcctgcgcgttgggtggtgaatggtattgaacgcagcggcgaagttaatgccaaaccgggtaccaaaagcggtgaccgtgtgggcatctgggtcgatagcgccggtcagctggtcgacgagccggcaccgccagcgcgtgcgatcgccgattctagacgcgcaattctgatccgcgttcgcaatgcgagctggcagcacgatattgatagcctgttttgcacccaacgtgagctcatgaccacggcgcgtgatatcatgaatgcgggtgtcacctgtgttggcgagcacgaaacgttgaccgcagcagcacagtacatgcgcgaacatgatatcggcgcattgccgatttgcggcgacgatgatcgtctgcacggtatgctgaccgaccgcgatatcgttatcaagggtctggccgcaggcttggacccgaacaccgcgaccgccggtgaactggcacgtgacagcatctattacgtcgacgcgaacgccagcattcaagagatgctgaacgtgatggaagagcatcaggtgcgtcgtgtcccggttatcagcgaacatcgtctggttggtatcgttaccgaagccgacatcgcacgtcacctgccggagcacgcgattgttcagttcgtgaaagcgatttgcagcccgatggcgttggcgtctaagcttttgctgggcctgagcaccattagcagcaaagcggatgacatcgactgggatgcgattgcgcagtgtgagagcggtggcaattgggcagcgaataccggcaatggcctgtacggcggtctgcagatctcccaggcgacgtgggacagcaatggtggcgtcggcagcccggctgccgcgtccccacaacaacagatcgaggtggcagataacattatgaaaacgcagggtccgggtgcttggccaaaatgctccagctgcagccagggtgacgcaccgctgggcagcctgacccacattctgacgttcctggcagcggaaaccggtggttgtagcggtagccgcgatgac

SEQ ID NO: 52 - DNA, 1689 bp, synthetic construct
  source 1..1689: mol_type = other DNA
  misc_feature 1..1689: note = Description of Artificial Sequence: Mycobacterium ESAT6-Rv1733c-Rv2626c-RpfD fusion protein (human optimized)
atgaccgagcagcagtggaacttcgccggcatcgaagctgccgctagcgccatccaaggcaacgtgaccagcatccacagcctgctggacgagggcaagcagagcctgaccaagctggctgctgcttggggcggatccggaagcgaagcctaccagggcgtgcagcagaagtgggacgccacagccaccgagctgaacaacgccctgcagaacctcgccagaaccatcagcgaggccggacaggctatggccagcacagagggcaatgtgaccggcatgttcgccttcgaaatcgccaccaccagggacagggaaggcgctaccatgatcaccttcaggctgaggctcccctgcaggaccatcctgagggtgttcagcaggaaccccctggtgaggggcaccgacagactggaagccgtgcaggacagcaggagccacgtgtatgcccaccaggctcagaccaggcaccctgctaccgccaccgtgatcgaccacgagggcgtgatcgactccaacaccaccgccaccagcgctcctcccagaaccaagatcacagtgcccgccaggtgggtggtgaacggcatcgagaggagcggcgaggtgaacgccaagcctggaaccaagagcggcgacagggtgggcatttgggtcgatagcgccggccagctggtggatgaacctgctccccctgccagagccatcgccgatagggccatcctgatcagggtgaggaacgccagctggcagcacgacatcgacagcctgttctgcacccaaaggcgatcgacaacagccagggacatcatgaacgccggcgtgacctgcgtgggagagcatgaaaccctcaccgccgccgcccaatacatgagggagcacgacatcggcgccctgcccatctgtggagacgacgacaggctgcacggcatgctgaccgacagggacatcgtgatcaagggcctggctgccggcctcgatcctaacaccgctacagccggcgagctggccagagacagcatctactacgtggacgccaacgccagcatccaggagatgctcaacgtgatggaggagcaccaggtgagaagggtgcctgtgatcagcgagcacaggctggtgggcatcgtgaccgaggccgatatcgctaggcacctgcccgagcacgccatcgtgcagttcgtgaaggccatctgcagccccatggctctggccagcggcgcgcccacccccggactcctcaccacagctggagctggcaggcccagagacagatgcgccaggatcgtgtgcaccgtgttcatcgagaccgccgtggtggctaccatgttcgtggccctgctgggcctgagcaccatcagcagcaaggccgacgacatcgactgggacgccatcgcccagtgtgaatccggcggaaactgggccgccaataccggcaatggcctgtacggcggcctgcagatcagccaggctacctgggactccaacggaggagtgggaagccctgccgctgcttcccctcagcagcagatcgaggtggccgacaacatcatgaagacccaaggccctggcgcctggcctaagtgttccagctgtagccagggcgatgctcctctgggcagcctgacccacatcctgacctttctcgccgccgagacaggcggatgtagcggaagcagggacgactaatgatag

SEQ ID NO: 53 - protein, 528 aa, synthetic construct
  SOURCE 1..528
  REGION 1..528: NOTE = Description of Artificial Sequence: ESAT6-Rv1733c-Rv2626c-RpfD(E. coli optimized)
MTEQQWNFAGIEAAASAIQGNVTSIHSLLDEGKQSLTKLAAAWGGSGSEAYQGVQQKWDATATELNNALQNLARTISEAGQAMASTEGNVTGMFAEFMIATTRDREGATMITFRLRLPCRTILRVFSRNPLVRGTDRLEAPGVQDSRSHVYAHQAQTRHPATATVIDHEGVIDSNTTATSAPPRTKITVPARWVVNGIERSGEVNAKPGTKSGDRVGIWVDSAGQLVDEPAPPARAIADSRRAILIRVRNASWQHDIDSLFCTQRELMTTARDIMNAGVTCVGEHETLTAAAQYMREHDIGALPICGDDDRLHGMLTDRDIVIKGLAAGLDPNTATAGELARDSIYYVDANASIQEMLNVMEEHQVRRVPVISEHRLVGIVTEADIARHLPEHAIVQFVKAICSPMALASKLLLGLSTISSKADDIDWDAIAQCESGGNWAANTGNGLYGGLQISQATWDSNGGVGSPAAASPQQQIEVADNIMKTQGPGAWPKCSSCSQGDAPLGSLTHILTFLAAETGGCSGSRDD

SEQ ID NO: 54 - protein, 559 aa, synthetic construct
  SOURCE 1..559
  REGION 1..559: NOTE = Description of Artificial Sequence: ESAT6-Rv1733c-Rv2626c-RpfD(human optimized)
MTEQQWNFAGIEAAASAIQGNVTSIHSLLDEGKQSLTKLAAAWGGSGSEAYQGVQQKWDATATELNNALNLARTISEAGQAMASTEGNVTGMFAFEIATTRDREGATMITFRLRLPCRTILRVFSRNPLVRGTDRLEAVQDSRSHVYAHQAQTRHPATATVIDHEGVIDSNTTATSAPPRTKITVPARWVVNGIERSGEVNAKPGTKSGDRVGIWVDSAGQLVDEPAPPARAIADRAILIRVRNASWQHDIDSLFCTQRRSTTARDIMNAGVTCVGEHETLTAAAQYMREHDIGALPICGDDDRLHGMLTDRDIVIKGLAAGLDPNTATAGELARDSIYYVDANASIQEMLNVMEEHQVRRVPVISEHRLVGIVTEADIARHLPEHAIVQFVKAICSPMALASGAPTPGLLTTAGAGRPRDRCARIVCTVFIETAVVATMFVALLGLSTISSKADDIDWDAIAQCESGGNWAANTGNGLYGGLQISQATWDSNGGVGSPAAASPQQQIEVADNIMKTQGPGAWPKCSSCSQGDAPLGSLTHILTFLAAETGGCSGSRDD

SEQ ID NO: 55 - DNA, 2421 bp, synthetic construct
  source 1..2421: mol_type = other DNA
  misc_feature 1..2421: note = Description of Artificial Sequence: Mycobacterium ESAT6-Rv1733c-Rv2626c-RpfB fusion protein
atgacagagcagcagtggaatttcgcgggtatcgaggccgcggcaagcgcaatccagggaaatgtcacgtccattcattccctccttgacgaggggaagcagtccctgaccaagctcgcagcggcctggggcggtagcggttcggaggcgtaccagggtgtccagcaaaaatgggacgccacggctaccgagctgaacaacgcgctgcagaacctggcgcggacgatcagcgaagccggtcaggcaatggcttcgaccgaaggcaacgtcactgggatgttcgcagaattcatgattgcgactacccgtgatcgtgagggcgcgaccatgatcacgttccgtctgcgtctgccgtgtcgcaccattttgcgcgtgttttcgcgtaacccgctggtccgcggtaccgaccgtctggaggccgttgtcatgctgctggcggttaccgtgagcctgctgacgatcccattcgcagcggcagctggcacggccgtccaagacagccgtagccatgtgtatgctcaccaggctcaaacccgtcacccggctactgccactgttatcgatcacgaaggcgtgattgactccaataccacggcaacctccgcaccgcctcgcaccaagattacggttcctgcgcgttgggtggtgaatggtattgaacgcagcggcgaagttaatgccaaaccgggtaccaaaagcggtgaccgtgtgggcatctgggtcgatagcgccggtcagctggtcgacgagccggcaccgccagcgcgtgcgatcgccgatgcggcgctggctgccctgggtctgtggctgagcgtggcagcggtcgccggtgcgttgctggcgctgacgcgcgcaattctgatccgcgttcgcaatgcgagctggcagcacgatattgatagcctgttttgcacccaacgtgagctcatgaccacggcgcgtgatatcatgaatgcgggtgtcacctgtgttggcgagcacgaaacgttgaccgcagcagcacagtacatgcgcgaacatgatatcggcgcattgccgatttgcggcgacgatgatcgtctgcacggtatgctgaccgaccgcgatatcgttatcaagggtctggccgcaggcttggacccgaacaccgcgaccgccggtgaactggcacgtgacagcatctattacgtcgacgcgaacgccagcattcaagagatgctgaacgtgatggaagagcatcaggtgcgtcgtgtcccggttatcagcgaacatcgtctggttggtatcgttaccgaagccgacatcgcacgtcacctgccggagcacgcgattgttcagttcgtgaaagcgatttgcagcccgatggcgttggcgtctcgtcaaaagggcgacacaaaatttattctaaatgcaaagcttgcatgcaaaacggtgacgttgaccgtcgacggaaccgcgatgcgggtgaccacgatgaaatcgcgggtgatcgacatcgtcgaagagaacgggttctcagtcgacgaccgcgacgacctgtatcccgcggccggcgtgcaggtccatgacgccgacaccatcgtgctgcggcgtagccgtccgctgcagatctcgctggatggtcacgacgctaagcaggtgtggacgaccgcgtcgacggtggacgaggcgctggcccaactcgcgatgaccgacacggcgccggccgcggcttctcgcgccagccgcgtcccgctgtccgggatggcgctaccggtcgtcagcgccaagacggtgcagctcaacgacggcgggttggtgcgcacggtgcacttgccggcccccaatgtcgcggggctgctgagtgcggccggcgtgccgctgttgcaaagcgaccacgtggtgcccgccgcgacggccccgatcgtcgaaggcatgcagatccaggtgacccgcaatcggatcaagaaggtcaccgagcggctgccgctgccgccgaacgcgcgtcgtgtcgaggacccggagatgaacatgagccgggaggtcgtcgaagacccgggggttccggggacccaggatgtgacgttcgcggtagctgaggtcaacggcgtcgagaccggccgtttgcccgtcgccaacgtcgtggtgaccccggcccacgaagccgtggtgcgggtgggcaccaagcccggtaccgaggtgcccccggtgatcgacggaagcatctgggacgcgatcgccggctgtgaggccggtggcaactgggcgatcaacaccggcaacgggtattacggtggtgtgcagtttgaccagggcacctgggaggccaacggcgggctgcggtatgcaccccgcgctgacctcgccacccgcgaagagcagatcgccgttgccgaggtgacccgactgcgtcaaggttggggcgcctggccggtatgtgctgcacgagcgggtgcgcgctga

SEQ ID NO: 56 - protein, 806 aa, synthetic construct
  SOURCE 1..806
  REGION 1..806: NOTE = Description of Artificial Sequence: ESAT6-Rv1733c-Rv2626c-RpfB
MTEQQWNFAGIEAAASAIQGNVTSIHSLLDEGKQSLTKLAAAWGGSGSEAYQGVQQKWDATATELNNALQNLARTISEAGQAMASTEGNVTGMFAEFMIATTRDREGATMITFRLRLPCRTILRVFSRNPLVRGTDRLEAVVMLLAVTVSLLTIPFAAAAGTAVQDSRSHVYAHQAQTRHPATATVIDHEGVIDSNTTATSAPPRTKITVPARWVVNGIERSGEVNAKPGTKSGDRVGIWVDSAGQLVDEPAPPARAIADAALAALGLWLSVAAVAGALLALTRAILIRVRNASWQHDIDSLFCTQRELMTTARDIMNAGVTCVGEHETLTAAAQYMREHDIGALPICGDDDRLHGMLTDRDIVIKGLAAGLDPNTATAGELARDSIYYVDANASIQEMLNVMEEHQVRRVPVISEHRLVGIVTEADIARHLPEHAIVQFVKAICSPMALASRQKGDTKFILNAKLACKTVTLTVDGTAMRVTTMKSRVIDIVEENGFSVDDRDDLYPAAGVQVHDADTIVLRRSRPLQISLDGHDAKQVWTTASTVDEALAQLAMTDTAPAAASRASRVPLSGMALPVVSAKTVQLNDGGLVRTVHLPAPNVAGLLSAAGVPLLQSDHVVPAATAPIVEGMQIQVTRNRIKKVTERLPLPPNARRVEDPEMNMSREVVEDPGVPGTQDVTFAVAEVNGVETGRLPVANVVVTPAHEAVVRVGTKPGTEVPPVIDGSIWDAIAGCEAGGNWAINTGNGYYGGVQFDQGTWEANGGLRYAPRADLATREEQIAVAEVTRLRQGWGAWPVCAARAGAR

SEQ ID NO: 57 - DNA, 2430 bp, synthetic construct
  source 1..2430: mol_type = other DNA
  misc_feature 1..2430: note = Description of Artificial Sequence: Mycobacterium RpfB-ESAT6-Rv1733c-Rv2626c fusion protein
atgaagcttgcatgcaaaacggtgacgttgaccgtcgacggaaccgcgatgcgggtgaccacgatgaaatcgcgggtgatcgacatcgtcgaagagaacgggttctcagtcgacgaccgcgacgacctgtatcccgcggccggcgtgcaggtccatgacgccgacaccatcgtgctgcggcgtagccgtccgctgcagatctcgctggatggtcacgacgctaagcaggtgtggacgaccgcgtcgacggtggacgaggcgctggcccaactcgcgatgaccgacacggcgccggccgcggcttctcgcgccagccgcgtcccgctgtccgggatggcgctaccggtcgtcagcgccaagacggtgcagctcaacgacggcgggttggtgcgcacggtgcacttgccggcccccaatgtcgcggggctgctgagtgcggccggcgtgccgctgttgcaaagcgaccacgtggtgcccgccgcgacggccccgatcgtcgaaggcatgcagatccaggtgacccgcaatcggatcaagaaggtcaccgagcggctgccgctgccgccgaacgcgcgtcgtgtcgaggacccggagatgaacatgagccgggaggtcgtcgaagacccgggggttccggggacccaggatgtgacgttcgcggtagctgaggtcaacggcgtcgagaccggccgtttgcccgtcgccaacgtcgtggtgaccccggcccacgaagccgtggtgcgggtgggcaccaagcccggtaccgaggtgcccccggtgatcgacggaagcatctgggacgcgatcgccggctgtgaggccggtggcaactgggcgatcaacaccggcaacgggtattacggtggtgtgcagtttgaccagggcacctgggaggccaacggcgggctgcggtatgcaccccgcgctgacctcgccacccgcgaagagcagatcgccgttgccgaggtgacccgactgcgtcaaggttggggcgcctggccggtatgtgctgcacgagcgggtgcgcgcggatccatgacagagcagcagtggaatttcgcgggtatcgaggccgcggcaagcgcaatccagggaaatgtcacgtccattcattccctccttgacgaggggaagcagtccctgaccaagctcgcagcggcctggggcggtagcggttcggaggcgtaccagggtgtccagcaaaaatgggacgccacggctaccgagctgaacaacgcgctgcagaacctggcgcggacgatcagcgaagccggtcaggcaatggcttcgaccgaaggcaacgtcactgggatgttcgcagaattcatgattgcgactacccgtgatcgtgagggcgcgaccatgatcacgttccgtctgcgtctgccgtgtcgcaccattttgcgcgtgttttcgcgtaacccgctggtccgcggtaccgaccgtctggaggccgttgtcatgctgctggcggttaccgtgagcctgctgacgatcccattcgcagcggcagctggcacggccgtccaagacagccgtagccatgtgtatgctcaccaggctcaaacccgtcacccggctactgccactgttatcgatcacgaaggcgtgattgactccaataccacggcaacctccgcaccgcctcgcaccaagattacggttcctgcgcgttgggtggtgaatggtattgaacgcagcggcgaagttaatgccaaaccgggtaccaaaagcggtgaccgtgtgggcatctgggtcgatagcgccggtcagctggtcgacgagccggcaccgccagcgcgtgcgatcgccgatgcggcgctggctgccctgggtctgtggctgagcgtggcagcggtcgccggtgcgttgctggcgctgacgcgcgcaattctgatccgcgttcgcaatgcgagctggcagcacgatattgatagcctgttttgcacccaacgtgagctcatgaccacggcgcgtgatatcatgaatgcgggtgtcacctgtgttggcgagcacgaaacgttgaccgcagcagcacagtacatgcgcgaacatgatatcggcgcattgccgatttgcggcgacgatgatcgtctgcacggtatgctgaccgaccgcgatatcgttatcaagggtctggccgcaggcttggacccgaacaccgcgaccgccggtgaactggcacgtgacagcatctattacgtcgacgcgaacgccagcattcaagagatgctgaacgtgatggaagagcatcaggtgcgtcgtgtcccggttatcagcgaacatcgtctggttggtatcgttaccgaagccgacatcgcacgtcacctgccggagcacgcgattgttcagttcgtgaaagcgatttgcagcccgatggcgttggcgtctcgtcaaaagggcgacacaaaatttattctaaatgcatga

SEQ ID NO: 58 - protein, 809 aa, synthetic construct
  SOURCE 1..809
  REGION 1..809: NOTE = Description of Artificial Sequence: RpfB-ESAT6-Rv1733c-Rv2626c
MKLACKTVTLTVDGTAMRVTTMKSRVIDIVEENGFSVDDRDDLYPAAGVQVHDADTIVLRRSRPLQISLDGHDAKQVWTTASTVDEALAQLAMTDTAPAAASRASRVPLSGMALPVVSAKTVQLNDGGLVRTVHLPAPNVAGLLSAAGVPLLQSDHVVPAATAPIVEGMQIQVTRNRIKKVTERLPLPPNARRVEDPEMNMSREVVEDPGVPGTQDVTFAVAEVNGVETGRLPVANVVVTPAHEAVVRVGTKPGTEVPPVIDGSIWDAIAGCEAGGNWAINTGNGYYGGVQFDQGTWEANGGLRYAPRADLATREEQIAVAEVTRLRQGWGAWPVCAARAGARGSMTEQQWNFAGIEAAASAIQGNVTSIHSLLDEGKQSLTKLAAAWGGSGSEAYQGVQQKWDATATELNNALQNLARTISEAGQAMASTEGNVTGMFAEFMIATTRDREGATMITFRLRLPCRTILRVFSRNPLVRGTDRLEAVVMLLAVTVSLLTIPFAAAAGTAVQDSRSHVYAHQAQTRHPATATVIDHEGVIDSNTTATSAPPRTKITVPARWVVNGIERSGEVNAKPGTKSGDRVGIWVDSAGQLVDEPAPPARAIADAALAALGLWLSVAAVAGALLALTRAILIRVRNASWQHDIDSLFCTQRELMTTARDIMNAGVTCVGEHETLTAAAQYMREHDIGALPICGDDDRLHGMLTDRDIVIKGLAAGLDPNTATAGELARDSIYYVDANASIQEMLNVMEEHQVRRVPVISEHRLVGIVTEADIARHLPEHAIVQFVKAICSPMALASRQKGDTKFILNA

SEQ ID NO: 59 - DNA, 2448 bp, synthetic construct
  source 1..2448: mol_type = other DNA
  misc_feature 1..2448: note = Description of Artificial Sequence: Mycobacterium Ag85B-ESAT6-Rv1733c-Rv2626c-RpfD fusion protein (E. coli optimized)
atgtttagccgtcctggcctgccagttgaatacctgcaagttccgagcccgtccatgggtcgtgacattaaggtgcagttccagagcggcggtaacaatagcccggctgtgtacctgctggacggtctgcgtgcgcaggatgattacaacggctgggacatcaataccccggcatttgagtggtattaccagtcgggtctgagcattgtgatgccggttggcggtcaaagcagcttctatagcgattggtacagcccggcatgcggcaaggctggttgccaaacctacaagtgggaaactttcttgaccagcgagctgccgcaatggttgagcgccaaccgtgcggtcaaaccgaccggtagcgctgctattggcctgtccatggccggcagcagcgcgatgatcttggcggcataccatccgcagcagtttatctacgccggtagcctgagcgcattgctggacccgagccaaggcatgggtccgagcctgattggtctggcaatgggtgacgcaggtggttacaaagcggccgatatgtggggcccatctagcgacccggcatgggagcgtaatgacccgacccagcaaattccgaaactggtggcgaataacacgcgcctgtgggtctactgtggcaatggtacgccgaacgagctgggtggcgcgaatatccctgcggagtttctggaaaactttgttcgcagcagcaacctgaaattccaggacgcgtataacgcagccggtggtcacaatgcggttttcaatttcccgccaaatggcactcatagctgggagtactggggtgcgcagttgaacgcaatgaaaggcgatctgcaatcctctctgggtgcgggcggatccatgacagagcagcagtggaatttcgcgggtatcgaggccgcggcaagcgcaatccagggaaatgtcacgtccattcattccctccttgacgaggggaagcagtccctgaccaagctcgcagcggcctggggcggtagcggttcggaggcgtaccagggtgtccagcaaaaatgggacgccacggctaccgagctgaacaacgcgctgcagaacctggcgcggacgatcagcgaagccggtcaggcaatggcttcgaccgaaggcaacgtcactgggatgttcgcagaattcatgattgcgactacccgtgatcgtgagggcgcgaccatgatcacgttccgtctgcgtctgccgtgtcgcaccattttgcgcgtgttttcgcgtaacccgctggtccgcggtaccgaccgtctggaggcccccggggtccaagacagccgtagccatgtgtatgctcaccaggctcaaacccgtcacccggctactgccactgttatcgatcacgaaggcgtgattgactccaataccacggcaacctccgcaccgcctcgcaccaagattacggttcctgcgcgttgggtggtgaatggtattgaacgcagcggcgaagttaatgccaaaccgggtaccaaaagcggtgaccgtgtgggcatctgggtcgatagcgccggtcagctggtcgacgagccggcaccgccagcgcgtgcgatcgccgattctagacgcgcaattctgatccgcgttcgcaatgcgagctggcagcacgatattgatagcctgttttgcacccaacgtgagctcatgaccacggcgcgtgatatcatgaatgcgggtgtcacctgtgttggcgagcacgaaacgttgaccgcagcagcacagtacatgcgcgaacatgatatcggcgcattgccgatttgcggcgacgatgatcgtctgcacggtatgctgaccgaccgcgatatcgttatcaagggtctggccgcaggcttggacccgaacaccgcgaccgccggtgaactggcacgtgacagcatctattacgtcgacgcgaacgccagcattcaagagatgctgaacgtgatggaagagcatcaggtgcgtcgtgtcccggttatcagcgaacatcgtctggttggtatcgttaccgaagccgacatcgcacgtcacctgccggagcacgcgattgttcagttcgtgaaagcgatttgcagcccgatggcgttggcgtctaagcttttgctgggcctgagcaccattagcagcaaagcggatgacatcgactgggatgcgattgcgcagtgtgagagcggtggcaattgggcagcgaataccggcaatggcctgtacggcggtctgcagatctcccaggcgacgtgggacagcaatggtggcgtcggcagcccggctgccgcgtccccacaacaacagatcgaggtggcagataacattatgaaaacgcagggtccgggtgcttggccaaaatgctccagctgcagccagggtgacgcaccgctgggcagcctgacccacattctgacgttcctggcagcggaaaccggtggttgtagcggtagccgcgatgac

SEQ ID NO: 60 - DNA, 2550 bp, synthetic construct
  source 1..2550: mol_type = other DNA
  misc_feature 1..2550: note = Description of Artificial Sequence: Mycobacterium Ag85B-ESAT6-Rv1733c-Rv2626c-RpfD fusion protein (human optimized)
atgttctccaggcccggcctgcctgtcgagtatctgcaggtcccctccccctccatgggcagagacatcaaggtgcagttccaatccggaggcaacaacagccccgccgtgtatctcctcgacggcctgagggctcaggacgactacaacggctgggacatcaacacccccgccttcgagtggtactaccagtccggactgagcatcgtcatgcccgtgggcggccagagctccttctacagcgactggtatagccctgcctgcggcaaagccggatgccagacctacaagtgggagacctttctgaccagcgaactgccccagtggctgtccgccaatagggccgtcaaacctaccggctccgctgccatcggactcagcatggccggaagctccgctatgatcctggccgcctaccacccccagcaatttatctacgctggcagcctgtccgctctgctggatcctagccaaggcatgggccctagcctcattggcctggccatgggcgatgctggcggctataaggccgccgatatgtggggccctagctccgatcctgcctgggagaggaatgaccccacccagcagatccccaagctggtggccaacaacacaaggctctgggtgtactgcggcaatggcacccccaacgaactgggcggagccaacattcccgccgagttcctggagaacttcgtcaggagcagcaacctgaagttccaggacgcctacaatgccgccggaggccacaacgctgtgttcaacttccctcccaacggcacccacagctgggagtattggggcgctcagctgaacgccatgaaaggcgacctccagagctccctgggagctggacccgggaccgagcagcagtggaacttcgccggcatcgaagctgccgctagcgccatccaaggcaacgtgaccagcatccacagcctgctggacgagggcaagcagagcctgaccaagctggctgctgcttggggcggatccggaagcgaagcctaccagggcgtgcagcagaagtgggacgccacagccaccgagctgaacaacgccctgcagaacctcgccagaaccatcagcgaggccggacaggctatggccagcacagagggcaatgtgaccggcatgttcgccttcgaaatcgccaccaccagggacagggaaggcgctaccatgatcaccttcaggctgaggctcccctgcaggaccatcctgagggtgttcagcaggaaccccctggtgaggggcaccgacagactggaagccgtgcaggacagcaggagccacgtgtatgcccaccaggctcagaccaggcaccctgctaccgccaccgtgatcgaccacgagggcgtgatcgactccaacaccaccgccaccagcgctcctcccagaaccaagatcacagtgcccgccaggtgggtggtgaacggcatcgagaggagcggcgaggtgaacgccaagcctggaaccaagagcggcgacagggtgggcatttgggtcgatagcgccggccagctggtggatgaacctgctccccctgccagagccatcgccgatagggccatcctgatcagggtgaggaacgccagctggcagcacgacatcgacagcctgttctgcacccaaaggcgatcgacaacagccagggacatcatgaacgccggcgtgacctgcgtgggagagcatgaaaccctcaccgccgccgcccaatacatgagggagcacgacatcggcgccctgcccatctgtggagacgacgacaggctgcacggcatgctgaccgacagggacatcgtgatcaagggcctggctgccggcctcgatcctaacaccgctacagccggcgagctggccagagacagcatctactacgtggacgccaacgccagcatccaggagatgctcaacgtgatggaggagcaccaggtgagaagggtgcctgtgatcagcgagcacaggctggtgggcatcgtgaccgaggccgatatcgctaggcacctgcccgagcacgccatcgtgcagttcgtgaaggccatctgcagccccatggctctggccagcggcgcgcccacccccggactcctcaccacagctggagctggcaggcccagagacagatgcgccaggatcgtgtgcaccgtgttcatcgagaccgccgtggtggctaccatgttcgtggccctgctgggcctgagcaccatcagcagcaaggccgacgacatcgactgggacgccatcgcccagtgtgaatccggcggaaactgggccgccaataccggcaatggcctgtacggcggcctgcagatcagccaggctacctgggactccaacggaggagtgggaagccctgccgctgcttcccctcagcagcagatcgaggtggccgacaacatcatgaagacccaaggccctggcgcctggcctaagtgttccagctgtagccagggcgatgctcctctgggcagcctgacccacatcctgacctttctcgccgccgagacaggcggatgtagcggaagcagggacgactaatgatag

SEQ ID NO: 61 - protein, 816 aa, synthetic construct
  SOURCE 1..816
  REGION 1..816: NOTE = Description of Artificial Sequence: Ag85B-ESAT6-Rv1733c-Rv2626c-RpfD(E. coli optimized)
MFSRPGLPVEYLQVPSPSMGRDIKVQFQSGGNNSPAVYLLDGLRAQDDYNGWDINTPAFEWYYQSGLSIVMPVGGQSSFYSDWYSPACGKAGCQTYKWETFLTSELPQWLSANRAVKPTGSAAIGLSMAGSSAMILAAYHPQQFIYAGSLSALLDPSQGMGPSLIGLAMGDAGGYKAADMWGPSSDPAWERNDPTQQIPKLVANNTRLWVYCGNGTPNELGGANIPAEFLENFVRSSNLKFQDAYNAAGGHNAVFNFPPNGTHSWEYWGAQLNAMKGDLQSSLGAGGSMTEQQWNFAGIEAAASAIQGNVTSIHSLLDEGKQSLTKLAAAWGGSGSEAYQGVQQKWDATATELNNALQNLARTISEAGQAMASTEGNVTGMFAEFMIATTRDREGATMITFRLRLPCRTILRVFSRNPLVRGTDRLEAPGVQDSRSHVYAHQAQTRHPATATVIDHEGVIDSNTTATSAPPRTKITVPARWVVNGIERSGEVNAKPGTKSGDRVGIWVDSAGQLVDEPAPPARAIADSRRAILIRVRNASWQHDIDSLFCTQRELMTTARDIMNAGVTCVGEHETLTAAAQYMREHDIGALPICGDDDRLHGMLTDRDIVIKGLAAGLDPNTATAGELARDSIYYVDANASIQEMLNVMEEHQVRRVPVISEHRLVGIVTEADIARHLPEHAIVQFVKAICSPMALASKLLLGLSTISSKADDIDWDAIAQCESGGNWAANTGNGLYGGLQISQATWDSNGGVGSPAAASPQQQIEVADNIMKTQGPGAWPKCSSCSQGDAPLGSLTHILTFLAAETGGCSGSRDD

SEQ ID NO: 62 - protein, 847 aa, synthetic construct
  SOURCE 1..847
  REGION 1..847: NOTE = Description of Artificial Sequence: Ag85B-ESAT6-Rv1733c-Rv2626c-RpfD(human optimized)
MFSRPGLPVEYLQVPSPSMGRDIKVQFQSGGNNSPAVYLLDGLRAQDDYNGWDINTPAFEWYYQSGLSIVMPVGGQSSFYSDWYSPACGKAGCQTYKWETFLTSELPQWLSANRAVKPTGSAAIGLSMAGSSAMILAAYHPQQFIYAGSLSALLDPSQGMGPSLIGLAMGDAGGYKAADMWGPSSDPAWERNDPTQQIPKLVANNTRLWVYCGNGTPNELGGANIPAEFLENFVRSSNLKFQDAYNAAGGHNAVFNFPPNGTHSWEYWGAQLNAMKGDLQSSLGAGPGTEQQWNFAGIEAAASAIQGNVTSIHSLLDEGKQSLTKLAAAWGGSGSEAYQGVQQKWDATATELNNALQNLARTISEAGQAMASTEGNVTGMFAFEIATTRDREGATMITFRLRLPCRTILRVFSRNPLVRGTDRLEAVQDSRSHVYAHQAQTRHPATATVIDHEGVIDSNTTATSAPPRTKITVPARWVVNGIERSGEVNAKPGTKSGDRVGIWVDSAGQLVDEPAPPARAIADRAILIRVRNASWQHDIDSLFCTQRRSTTARDIMNAGVTCVGEHETLTAAAQYMREHDIGALPICGDDDRLHGMLTDRDIVIKGLAAGLDPNTATAGELARDSIYYVDANASIQEMLNVMEEHQVRRVPVISEHRLVGIVTEADIARHLPEHAIVQFVKAICSPMALASGAPTPGLLTTAGAGRPRDRCARIVCTVFIETAVVATMFVALLGLSTISSKADDIDWDAIAQCESGGNWAANTGNGLYGGLQISQATWDSNGGVGSPAAASPQQQIEVADNIMKTQGPGAWPKCSSCSQGDAPLGSLTHILTFLAAETGGCSGSRDD

SEQ ID NO: 63 - DNA, 2499 bp, synthetic construct
  source 1..2499: mol_type = other DNA
  misc_feature 1..2499: note = Description of Artificial Sequence: Mycobacterium PPE51-Rv1733c-Rv2628c-RpfD fusion protein
atggattttgcgctgctgccgccggaagtgaacagcgcgcgcatgtataccggcccgggcgcgggcagcctgctggcggcggcgggcggctgggatagcctggcggcggaactggcgaccaccgcggaagcgtatggcagcgtgctgagcggcctggcggcgctgcattggcgcggcccggcggcggaaagcatggcggtgaccgcggcgccgtatattggctggctgtataccaccgcggaaaaaacccagcagaccgcgattcaggcgcgcgcggcggcgctggcgtttgaacaggcgtatgcgatgaccctgccgccgccggtggtggcggcgaaccgcattcagctgctggcgctgattgcgaccaacttttttggccagaacaccgcggcgattgcggcgaccgaagcgcagtatgcggaaatgtgggcgcaggatgcggcggcgatgtatggctatgcgaccgcgagcgcggcggcggcgctgctgaccccgtttagcccgccgcgccagaccaccaacccggcgggcctgaccgcgcaggcggcggcggtgagccaggcgaccgatccgctgagcctgctgattgaaaccgtgacccaggcgctgcaggcgctgaccattccgagctttattccggaagattttacctttctggatgcgatttttgcgggctatgcgaccgtgggcgtgacccaggatgtggaaagctttgtggcgggcaccattggcgcggaaagcaacctgggcctgctgaacgtgggcgatgaaaacccggcggaagtgaccccgggcgattttggcattggcgaactggtgagcgcgaccagcccgggcggcggcgtgagcgcgagcggcgcgggcggcgcggcgagcgtgggcaacaccgtgctggcgagcgtgggccgcgcgaacagcattggccagctgagcgtgccgccgagctgggcggcgccgagcacccgcccggtgagcgcgctgagcccggcgggcctgaccaccctgccgggcaccgatgtggcggaacatggcatgccgggcgtgccgggcgtgccggtggcggcgggccgcgcgagcggcgtgctgccgcgctatggcgtgcgcctgaccgtgatggcgcatccgccggcggcgggcgaattcatgattgcgactacccgtgatcgtgagggcgcgaccatgatcacgttccgtctgcgtctgccgtgtcgcaccattttgcgcgtgttttcgcgtaacccgctggtccgcggtaccgaccgtctggaggccgttgtcatgctgctggcggttaccgtgagcctgctgacgatcccattcgcagcggcagctggcacggccgtccaagacagccgtagccatgtgtatgctcaccaggctcaaacccgtcacccggctactgccactgttatcgatcacgaaggcgtgattgactccaataccacggcaacctccgcaccgcctcgcaccaagattacggttcctgcgcgttgggtggtgaatggtattgaacgcagcggcgaagttaatgccaaaccgggtaccaaaagcggtgaccgtgtgggcatctgggtcgatagcgccggtcagctggtcgacgagccggcaccgccagcgcgtgcgatcgccgatgcggcgctggctgccctgggtctgtggctgagcgtggcagcggtcgccggtgcgttgctggcgctgacgcgcgcaattctgatccgcgttcgcaatgcgagctggcagcacgatattgatagcctgttttgcacccaacgtgagctcatgtccacgcaacgaccgaggcactccggtattcgggctgttggcccctacgcatgggccggccgatgtggtcggataggcaggtggggggtgcaccaggaggcgatgatgaatctagcgatatggcacccgcgcaaggtgcaatccgccaccatctatcaggtgaccgatcgctcgcacgacgggcgcacagcacgggtgcctggtgacgagatcactagcaccgtgtccggttggttgtcggagttgggcacccaaagcccgttggccgatgagcttgcgcgtgcggtgcggatcggcgactggcccgctgcgtacgcaatcggtgagcacctgtccgttgagattgccgttgcggtcaagcttttgctgggcctgagcaccattagcagcaaagcggatgacatcgactgggatgcgattgcgcagtgtgagagcggtggcaattgggcagcgaataccggcaatggcctgtacggcggtctgcagatctcccaggcgacgtgggacagcaatggtggcgtcggcagcccggctgccgcgtccccacaacaacagatcgaggtggcagataacattatgaaaacgcagggtccgggtgcttggccaaaatgctccagctgcagccagggtgacgcaccgctgggcagcctgacccacattctgacgttcctggcagcggaaaccggtggttgtagcggtagccgcgatgactga

SEQ ID NO: 64 - protein, 834 aa, synthetic construct
  SOURCE 1..834
  REGION 1..834: NOTE = Description of Artificial Sequence: PPE51-Rv1733c-Rv2628c-RpfD
MDFALLPPEVNSARMYTGPGAGSLLAAAGGWDSLAAELATTAEAYGSVLSGLAALHWRGPAAESMAVTAAPYIGWLYTTAEKTQQTAIQARAAALAFEQAYAMTLPPPVVAANRIQLLALIATNFFGQNTAAIAATEAQYAEMWAQDAAAMYGYATASAAAALLTPFSPPRQTTNPAGLTAQAAAVSQATDPLSLLIETVTQALQALTIPSFIPEDFTFLDAIFAGYATVGVTQDVESFVAGTIGAESNLGLLNVGDENPAEVTPGDFGIGELVSATSPGGGVSASGAGGAASVGNTVLASVGRANSIGQLSVPPSWAAPSTRPVSALSPAGLTTLPGTDVAEHGMPGVPGVPVAAGRASGVLPRYGVRLTVMAHPPAAGEFEFMIATTRDREGATMITFRLRLPCRTILRVFSRNPLVRGTDRLEAVVMLLAVTVSLLTIPFAAAAGTAVQDSRSHVYAHQAQTRHPATATVIDHEGVIDSNTTATSAPPRTKITVPARWVVNGIERSGEVNAKPGTKSGDRVGIWVDSAGQLVDEPAPPARAIADAALAALGLWLSVAAVAGALLALTRAILIRVRNASWQHDIDSLFCTQRELMSTQRPRHSGIRAVGPYAWAGRCGRIGRWGVHQEAMMNLAIWHPRKVQSATIYQVTDRSHDGRTARVPGDEITSTVSGWLSELGTQSPLADELARAVRIGDWPAAYAIGEHLSVEIAVAVKLLLGLSTISSKADDIDWDAIAQCESGGNWAANTGNGLYGGLQISQATWDSNGGVGSPAAASPQQQIEVADNIMKTQGPGAWPKCSSCSQGDAPLGSLTHILTFLAAETGGCSGSRDD

SEQ ID NO: 65 - DNA, 3171 bp, synthetic construct
  source 1..3171: mol_type = other DNA
  misc_feature 1..3171: note = Description of Artificial Sequence: Mycobacterium PPE51-Rv1733c-Rv2628c-RpfB fusion protein
atggattttgcgctgctgccgccggaagtgaacagcgcgcgcatgtataccggcccgggcgcgggcagcctgctggcggcggcgggcggctgggatagcctggcggcggaactggcgaccaccgcggaagcgtatggcagcgtgctgagcggcctggcggcgctgcattggcgcggcccggcggcggaaagcatggcggtgaccgcggcgccgtatattggctggctgtataccaccgcggaaaaaacccagcagaccgcgattcaggcgcgcgcggcggcgctggcgtttgaacaggcgtatgcgatgaccctgccgccgccggtggtggcggcgaaccgcattcagctgctggcgctgattgcgaccaacttttttggccagaacaccgcggcgattgcggcgaccgaagcgcagtatgcggaaatgtgggcgcaggatgcggcggcgatgtatggctatgcgaccgcgagcgcggcggcggcgctgctgaccccgtttagcccgccgcgccagaccaccaacccggcgggcctgaccgcgcaggcggcggcggtgagccaggcgaccgatccgctgagcctgctgattgaaaccgtgacccaggcgctgcaggcgctgaccattccgagctttattccggaagattttacctttctggatgcgatttttgcgggctatgcgaccgtgggcgtgacccaggatgtggaaagctttgtggcgggcaccattggcgcggaaagcaacctgggcctgctgaacgtgggcgatgaaaacccggcggaagtgaccccgggcgattttggcattggcgaactggtgagcgcgaccagcccgggcggcggcgtgagcgcgagcggcgcgggcggcgcggcgagcgtgggcaacaccgtgctggcgagcgtgggccgcgcgaacagcattggccagctgagcgtgccgccgagctgggcggcgccgagcacccgcccggtgagcgcgctgagcccggcgggcctgaccaccctgccgggcaccgatgtggcggaacatggcatgccgggcgtgccgggcgtgccggtggcggcgggccgcgcgagcggcgtgctgccgcgctatggcgtgcgcctgaccgtgatggcgcatccgccggcggcgggcgaattcatgattgcgactacccgtgatcgtgagggcgcgaccatgatcacgttccgtctgcgtctgccgtgtcgcaccattttgcgcgtgttttcgcgtaacccgctggtccgcggtaccgaccgtctggaggccgttgtcatgctgctggcggttaccgtgagcctgctgacgatcccattcgcagcggcagctggcacggccgtccaagacagccgtagccatgtgtatgctcaccaggctcaaacccgtcacccggctactgccactgttatcgatcacgaaggcgtgattgactccaataccacggcaacctccgcaccgcctcgcaccaagattacggttcctgcgcgttgggtggtgaatggtattgaacgcagcggcgaagttaatgccaaaccgggtaccaaaagcggtgaccgtgtgggcatctgggtcgatagcgccggtcagctggtcgacgagccggcaccgccagcgcgtgcgatcgccgatgcggcgctggctgccctgggtctgtggctgagcgtggcagcggtcgccggtgcgttgctggcgctgacgcgcgcaattctgatccgcgttcgcaatgcgagctggcagcacgatattgatagcctgttttgcacccaacgtgagctcatgtccacgcaacgaccgaggcactccggtattcgggctgttggcccctacgcatgggccggccgatgtggtcggataggcaggtggggggtgcaccaggaggcgatgatgaatctagcgatatggcacccgcgcaaggtgcaatccgccaccatctatcaggtgaccgatcgctcgcacgacgggcgcacagcacgggtgcctggtgacgagatcactagcaccgtgtccggttggttgtcggagttgggcacccaaagcccgttggccgatgagcttgcgcgtgcggtgcggatcggcgactggcccgctgcgtacgcaatcggtgagcacctgtccgttgagattgccgttgcggtcaagcttgcatgcaaaacggtgacgttgaccgtcgacggaaccgcgatgcgggtgaccacgatgaaatcgcgggtgatcgacatcgtcgaagagaacgggttctcagtcgacgaccgcgacgacctgtatcccgcggccggcgtgcaggtccatgacgccgacaccatcgtgctgcggcgtagccgtccgctgcagatctcgctggatggtcacgacgctaagcaggtgtggacgaccgcgtcgacggtggacgaggcgctggcccaactcgcgatgaccgacacggcgccggccgcggcttctcgcgccagccgcgtcccgctgtccgggatggcgctaccggtcgtcagcgccaagacggtgcagctcaacgacggcgggttggtgcgcacggtgcacttgccggcccccaatgtcgcggggctgctgagtgcggccggcgtgccgctgttgcaaagcgaccacgtggtgcccgccgcgacggccccgatcgtcgaaggcatgcagatccaggtgacccgcaatcggatcaagaaggtcaccgagcggctgccgctgccgccgaacgcgcgtcgtgtcgaggacccggagatgaacatgagccgggaggtcgtcgaagacccgggggttccggggacccaggatgtgacgttcgcggtagctgaggtcaacggcgtcgagaccggccgtttgcccgtcgccaacgtcgtggtgaccccggcccacgaagccgtggtgcgggtgggcaccaagcccggtaccgaggtgcccccggtgatcgacggaagcatctgggacgcgatcgccggctgtgaggccggtggcaactgggcgatcaacaccggcaacgggtattacggtggtgtgcagtttgaccagggcacctgggaggccaacggcgggctgcggtatgcaccccgcgctgacctcgccacccgcgaagagcagatcgccgttgccgaggtgacccgactgcgtcaaggttggggcgcctggccggtatgtgctgcacgagcgggtgcgcgctga

SEQ ID NO: 66 - protein, 1056 aa, synthetic construct
  SOURCE 1..1056
  REGION 1..1056: NOTE = Description of Artificial Sequence: PPE51-Rv1733c-Rv2628c-RpfB
MDFALLPPEVNSARMYTGPGAGSLLAAAGGWDSLAAELATTAEAYGSVLSGLAALHWRGPAAESMAVTAAPYIGWLYTTAEKTQQTAIQARAAALAFEQAYAMTLPPPVVAANRIQLLALIATNFFGQNTAAIAATEAQYAEMWAQDAAAMYGYATASAAAALLTPFSPPRQTTNPAGLTAQAAAVSQATDPLSLLIETVTQALQALTIPSFIPEDFTFLDAIFAGYATVGVTQDVESFVAGTIGAESNLGLLNVGDENPAEVTPGDFGIGELVSATSPGGGVSASGAGGAASVGNTVLASVGRANSIGQLSVPPSWAAPSTRPVSALSPAGLTTLPGTDVAEHGMPGVPGVPVAAGRASGVLPRYGVRLTVMAHPPAAGEFMIATTRDREGATMITFRLRLPCRTILRVFSRNPLVRGTDRLEAVVMLLAVTVSLLTIPFAAAAGTAVQDSRSHVYAHQAQTRHPATATVIDHEGVIDSNTTATSAPPRTKITVPARWVVNGIERSGEVNAKPGTKSGDRVGIWVDSAGQLVDEPAPPARAIADAALAALGLWLSVAAVAGALLALTRAILIRVRNASWQHDIDSLFCTQRELMSTQRPRHSGIRAVGPYAWAGRCGRIGRWGVHQEAMMNLAIWHPRKVQSATIYQVTDRSHDGRTARVPGDEITSTVSGWLSELGTQSPLADELARAVRIGDWPAAYAIGEHLSVEIAVAVKLACKTVTLTVDGTAMRVTTMKSRVIDIVEENGFSVDDRDDLYPAAGVQVHDADTIVLRRSRPLQISLDGHDAKQVWTTASTVDEALAQLAMTDTAPAAASRASRVPLSGMALPVVSAKTVQLNDGGLVRTVHLPAPNVAGLLSAAGVPLLQSDHVVPAATAPIVEGMQIQVTRNRIKKVTERLPLPPNARRVEDPEMNMSREVVEDPGVPGTQDVTFAVAEVNGVETGRLPVANVVVTPAHEAVVRVGTKPGTEVPPVIDGSIWDAIAGCEAGGNWAINTGNGYYGGVQFDQGTWEANGGLRYAPRADLATREEQIAVAEVTRLRQGWGAWPVCAARAGAR

SEQ ID NO: 67 - DNA, 2433 bp, synthetic construct
  source 1..2433: mol_type = other DNA
  misc_feature 1..2433: note = Description of Artificial Sequence: Mycobacterium Rv3407-Rv1733c-Rv2626c-RpfB fusion protein
atgcgtgcgactgtgggtctggttgaggcgattggcattcgcgagctgcgccaacatgccagccgttacttggctcgtgtcgaggcgggtgaagaactgggcgtgacgaataagggtcgtctggtcgcccgtctgattccggttcaggcagctgagcgttctcgcgaggcgctgattgaatccggcgtcctgatcccggctcgccgtccgcaaaacctgctggacgtgacggcggagccagctcgtggtcgcaaacgcacgctgtctgatgtcctgaacgaaatgcgcgacgagcaggaattcatgattgcgactacccgtgatcgtgagggcgcgaccatgatcacgttccgtctgcgtctgccgtgtcgcaccattttgcgcgtgttttcgcgtaacccgctggtccgcggtaccgaccgtctggaggccgttgtcatgctgctggcggttaccgtgagcctgctgacgatcccattcgcagcggcagctggcacggccgtccaagacagccgtagccatgtgtatgctcaccaggctcaaacccgtcacccggctactgccactgttatcgatcacgaaggcgtgattgactccaataccacggcaacctccgcaccgcctcgcaccaagattacggttcctgcgcgttgggtggtgaatggtattgaacgcagcggcgaagttaatgccaaaccgggtaccaaaagcggtgaccgtgtgggcatctgggtcgatagcgccggtcagctggtcgacgagccggcaccgccagcgcgtgcgatcgccgatgcggcgctggctgccctgggtctgtggctgagcgtggcagcggtcgccggtgcgttgctggcgctgacgcgcgcaattctgatccgcgttcgcaatgcgagctggcagcacgatattgatagcctgttttgcacccaacgtgagctcatgaccacggcgcgtgatatcatgaatgcgggtgtcacctgtgttggcgagcacgaaacgttgaccgcagcagcacagtacatgcgcgaacatgatatcggcgcattgccgatttgcggcgacgatgatcgtctgcacggtatgctgaccgaccgcgatatcgttatcaagggtctggccgcaggcttggacccgaacaccgcgaccgccggtgaactggcacgtgacagcatctattacgtcgacgcgaacgccagcattcaagagatgctgaacgtgatggaagagcatcaggtgcgtcgtgtcccggttatcagcgaacatcgtctggttggtatcgttaccgaagccgacatcgcacgtcacctgccggagcacgcgattgttcagttcgtgaaagcgatttgcagcccgatggcgttggcgtctcgtcaaaagggcgacacaaaatttattctaaatgcaaagcttgcatgcaaaacggtgacgttgaccgtcgacggaaccgcgatgcgggtgaccacgatgaaatcgcgggtgatcgacatcgtcgaagagaacgggttctcagtcgacgaccgcgacgacctgtatcccgcggccggcgtgcaggtccatgacgccgacaccatcgtgctgcggcgtagccgtccgctgcagatctcgctggatggtcacgacgctaagcaggtgtggacgaccgcgtcgacggtggacgaggcgctggcccaactcgcgatgaccgacacggcgccggccgcggcttctcgcgccagccgcgtcccgctgtccgggatggcgctaccggtcgtcagcgccaagacggtgcagctcaacgacggcgggttggtgcgcacggtgcacttgccggcccccaatgtcgcggggctgctgagtgcggccggcgtgccgctgttgcaaagcgaccacgtggtgcccgccgcgacggccccgatcgtcgaaggcatgcagatccaggtgacccgcaatcggatcaagaaggtcaccgagcggctgccgctgccgccgaacgcgcgtcgtgtcgaggacccggagatgaacatgagccgggaggtcgtcgaagacccgggggttccggggacccaggatgtgacgttcgcggtagctgaggtcaacggcgtcgagaccggccgtttgcccgtcgccaacgtcgtggtgaccccggcccacgaagccgtggtgcgggtgggcaccaagcccggtaccgaggtgcccccggtgatcgacggaagcatctgggacgcgatcgccggctgtgaggccggtggcaactgggcgatcaacaccggcaacgggtattacggtggtgtgcagtttgaccagggcacctgggaggccaacggcgggctgcggtatgcaccccgcgctgacctcgccacccgcgaagagcagatcgccgttgccgaggtgacccgactgcgtcaaggttggggcgcctggccggtatgtgctgcacgagcgggtgcgcgctga

SEQ ID NO: 68 - protein, 810 aa, synthetic construct
  SOURCE 1..810
  REGION 1..810: NOTE = Description of Artificial Sequence: Rv3407-Rv1733c-Rv2626c-RpfB
MRATVGLVEAIGIRELRQHASRYLARVEAGEELGVTNKGRLVARLIPVQAAERSREALIESGVLIPARRPQNLLDVTAEPARGRKRTLSDVLNEMRDEQEFMIATTRDREGATMITFRLRLPCRTILRVFSRNPLVRGTDRLEAVVMLLAVTVSLLTIPFAAAAGTAVQDSRSHVYAHQAQTRHPATATVIDHEGVIDSNTTATSAPPRTKITVPARWVVNGIERSGEVNAKPGTKSGDRVGIWVDSAGQLVDEPAPPARAIADAALAALGLWLSVAAVAGALLALTRAILIRVRNASWQHDIDSLFCTQRELMTTARDIMNAGVTCVGEHETLTAAAQYMREHDIGALPICGDDDRLHGMLTDRDIVIKGLAAGLDPNTATAGELARDSIYYVDANASIQEMLNVMEEHQVRRVPVISEHRLVGIVTEADIARHLPEHAIVQFVKAICSPMALASRQKGDTKFILNAKLACKTVTLTVDGTAMRVTTMKSRVIDIVEENGFSVDDRDDLYPAAGVQVHDADTIVLRRSRPLQISLDGHDAKQVWTTASTVDEALAQLAMTDTAPAAASRASRVPLSGMALPVVSAKTVQLNDGGLVRTVHLPAPNVAGLLSAAGVPLLQSDHVVPAATAPIVEGMQIQVTRNRIKKVTERLPLPPNARRVEDPEMNMSREVVEDPGVPGTQDVTFAVAEVNGVETGRLPVANVVVTPAHEAVVRVGTKPGTEVPPVIDGSIWDAIAGCEAGGNWAINTGNGYYGGVQFDQGTWEANGGLRYAPRADLATREEQIAVAEVTRLRQGWGAWPVCAARAGAR

SEQ ID NO: 69 - DNA, 1761 bp, synthetic construct
  source 1..1761: mol_type = other DNA
  misc_feature 1..1761: note = Description of Artificial Sequence: Mycobacterium Rv3407-Rv1733c-Rv2626c-RpfD fusion protein
atgcgtgcgactgtgggtctggttgaggcgattggcattcgcgagctgcgccaacatgccagccgttacttggctcgtgtcgaggcgggtgaagaactgggcgtgacgaataagggtcgtctggtcgcccgtctgattccggttcaggcagctgagcgttctcgcgaggcgctgattgaatccggcgtcctgatcccggctcgccgtccgcaaaacctgctggacgtgacggcggagccagctcgtggtcgcaaacgcacgctgtctgatgtcctgaacgaaatgcgcgacgagcaggaattcatgattgcgactacccgtgatcgtgagggcgcgaccatgatcacgttccgtctgcgtctgccgtgtcgcaccattttgcgcgtgttttcgcgtaacccgctggtccgcggtaccgaccgtctggaggccgttgtcatgctgctggcggttaccgtgagcctgctgacgatcccattcgcagcggcagctggcacggccgtccaagacagccgtagccatgtgtatgctcaccaggctcaaacccgtcacccggctactgccactgttatcgatcacgaaggcgtgattgactccaataccacggcaacctccgcaccgcctcgcaccaagattacggttcctgcgcgttgggtggtgaatggtattgaacgcagcggcgaagttaatgccaaaccgggtaccaaaagcggtgaccgtgtgggcatctgggtcgatagcgccggtcagctggtcgacgagccggcaccgccagcgcgtgcgatcgccgatgcggcgctggctgccctgggtctgtggctgagcgtggcagcggtcgccggtgcgttgctggcgctgacgcgcgcaattctgatccgcgttcgcaatgcgagctggcagcacgatattgatagcctgttttgcacccaacgtgagctcatgaccacggcgcgtgatatcatgaatgcgggtgtcacctgtgttggcgagcacgaaacgttgaccgcagcagcacagtacatgcgcgaacatgatatcggcgcattgccgatttgcggcgacgatgatcgtctgcacggtatgctgaccgaccgcgatatcgttatcaagggtctggccgcaggcttggacccgaacaccgcgaccgccggtgaactggcacgtgacagcatctattacgtcgacgcgaacgccagcattcaagagatgctgaacgtgatggaagagcatcaggtgcgtcgtgtcccggttatcagcgaacatcgtctggttggtatcgttaccgaagccgacatcgcacgtcacctgccggagcacgcgattgttcagttcgtgaaagcgatttgcagcccgatggcgttggcgtctcgtcaaaagggcgacacaaaatttattctaaatgcaaagcttttgctgggcctgagcaccattagcagcaaagcggatgacatcgactgggatgcgattgcgcagtgtgagagcggtggcaattgggcagcgaataccggcaatggcctgtacggcggtctgcagatctcccaggcgacgtgggacagcaatggtggcgtcggcagcccggctgccgcgtccccacaacaacagatcgaggtggcagataacattatgaaaacgcagggtccgggtgcttggccaaaatgctccagctgcagccagggtgacgcaccgctgggcagcctgacccacattctgacgttcctggcagcggaaaccggtggttgtagcggtagccgcgatgactga

SEQ ID NO: 70 - protein, 586 aa, synthetic construct
  SOURCE 1..586
  REGION 1..586: NOTE = Description of Artificial Sequence: Rv3407-Rv1733c-Rv2626c-RpfD
MRATVGLVEAIGIRELRQHASRYLARVEAGEELGVTNKGRLVARLIPVQAAERSREALIESGVLIPARRPQNLLDVTAEPARGRKRTLSDVLNEMRDEQEFMIATTRDREGATMITFRLRLPCRTILRVFSRNPLVRGTDRLEAVVMLLAVTVSLLTIPFAAAAGTAVQDSRSHVYAHQAQTRHPATATVIDHEGVIDSNTTATSAPPRTKITVPARWVVNGIERSGEVNAKPGTKSGDRVGIWVDSAGQLVDEPAPPARAIADAALAALGLWLSVAAVAGALLALTRAILIRVRNASWQHDIDSLFCTQRELMTTARDIMNAGVTCVGEHETLTAAAQYMREHDIGALPICGDDDRLHGMLTDRDIVIKGLAAGLDPNTATAGELARDSIYYVDANASIQEMLNVMEEHQVRRVPVISEHRLVGIVTEADIARHLPEHAIVQFVKAICSPMALASRQKGDTKFILNAKLLLGLSTISSKADDIDWDAIAQCESGGNWAANTGNGLYGGLQISQATWDSNGGVGSPAAASPQQQIEVADNIMKTQGPGAWPKCSSCSQGDAPLGSLTHILTFLAAETGGCSGSRDD

SEQ ID NO: 71 - DNA, 2895 bp, synthetic construct
  source 1..2895: mol_type = other DNA
  misc_feature 1..2895: note = Description of Artificial Sequence: Mycobacterium PPE51-Rv1733c-Rv2626c-RpfD fusion protein
atggattttgcgctgctgccgccggaagtgaacagcgcgcgcatgtataccggcccgggcgcgggcagcctgctggcggcggcgggcggctgggatagcctggcggcggaactggcgaccaccgcggaagcgtatggcagcgtgctgagcggcctggcggcgctgcattggcgcggcccggcggcggaaagcatggcggtgaccgcggcgccgtatattggctggctgtataccaccgcggaaaaaacccagcagaccgcgattcaggcgcgcgcggcggcgctggcgtttgaacaggcgtatgcgatgaccctgccgccgccggtggtggcggcgaaccgcattcagctgctggcgctgattgcgaccaacttttttggccagaacaccgcggcgattgcggcgaccgaagcgcagtatgcggaaatgtgggcgcaggatgcggcggcgatgtatggctatgcgaccgcgagcgcggcggcggcgctgctgaccccgtttagcccgccgcgccagaccaccaacccggcgggcctgaccgcgcaggcggcggcggtgagccaggcgaccgatccgctgagcctgctgattgaaaccgtgacccaggcgctgcaggcgctgaccattccgagctttattccggaagattttacctttctggatgcgatttttgcgggctatgcgaccgtgggcgtgacccaggatgtggaaagctttgtggcgggcaccattggcgcggaaagcaacctgggcctgctgaacgtgggcgatgaaaacccggcggaagtgaccccgggcgattttggcattggcgaactggtgagcgcgaccagcccgggcggcggcgtgagcgcgagcggcgcgggcggcgcggcgagcgtgggcaacaccgtgctggcgagcgtgggccgcgcgaacagcattggccagctgagcgtgccgccgagctgggcggcgccgagcacccgcccggtgagcgcgctgagcccggcgggcctgaccaccctgccgggcaccgatgtggcggaacatggcatgccgggcgtgccgggcgtgccggtggcggcgggccgcgcgagcggcgtgctgccgcgctatggcgtgcgcctgaccgtgatggcgcatccgccggcggcgggcgaatttatgacagagcagcagtggaatttcgcgggtatcgaggccgcggcaagcgcaatccagggaaatgtcacgtccattcattccctccttgacgaggggaagcagtccctgaccaagctcgcagcggcctggggcggtagcggttcggaggcgtaccagggtgtccagcaaaaatgggacgccacggctaccgagctgaacaacgcgctgcagaacctggcgcggacgatcagcgaagccggtcaggcaatggcttcgaccgaaggcaacgtcactgggatgttcgcagaattcatgattgcgactacccgtgatcgtgagggcgcgaccatgatcacgttccgtctgcgtctgccgtgtcgcaccattttgcgcgtgttttcgcgtaacccgctggtccgcggtaccgaccgtctggaggccgttgtcatgctgctggcggttaccgtgagcctgctgacgatcccattcgcagcggcagctggcacggccgtccaagacagccgtagccatgtgtatgctcaccaggctcaaacccgtcacccggctactgccactgttatcgatcacgaaggcgtgattgactccaataccacggcaacctccgcaccgcctcgcaccaagattacggttcctgcgcgttgggtggtgaatggtattgaacgcagcggcgaagttaatgccaaaccgggtaccaaaagcggtgaccgtgtgggcatctgggtcgatagcgccggtcagctggtcgacgagccggcaccgccagcgcgtgcgatcgccgatgcggcgctggctgccctgggtctgtggctgagcgtggcagcggtcgccggtgcgttgctggcgctgacgcgcgcaattctgatccgcgttcgcaatgcgagctggcagcacgatattgatagcctgttttgcacccaacgtgagctcatgaccacggcgcgtgatatcatgaatgcgggtgtcacctgtgttggcgagcacgaaacgttgaccgcagcagcacagtacatgcgcgaacatgatatcggcgcattgccgatttgcggcgacgatgatcgtctgcacggtatgctgaccgaccgcgatatcgttatcaagggtctggccgcaggcttggacccgaacaccgcgaccgccggtgaactggcacgtgacagcatctattacgtcgacgcgaacgccagcattcaagagatgctgaacgtgatggaagagcatcaggtgcgtcgtgtcccggttatcagcgaacatcgtctggttggtatcgttaccgaagccgacatcgcacgtcacctgccggagcacgcgattgttcagttcgtgaaagcgatttgcagcccgatggcgttggcgtctcgtcaaaagggcgacacaaaatttattctaaatgcaaagcttttgctgggcctgagcaccattagcagcaaagcggatgacatcgactgggatgcgattgcgcagtgtgagagcggtggcaattgggcagcgaataccggcaatggcctgtacggcggtctgcagatctcccaggcgacgtgggacagcaatggtggcgtcggcagcccggctgccgcgtccccacaacaacagatcgaggtggcagataacattatgaaaacgcagggtccgggtgcttggccaaaatgctccagctgcagccagggtgacgcaccgctgggcagcctgacccacattctgacgttcctggcagcggaaaccggtggttgtagcggtagccgcgatgactga

SEQ ID NO: 72 - protein, 870 aa, synthetic construct
  SOURCE 1..870
  REGION 1..870: NOTE = Description of Artificial Sequence: PPE51-Rv1733c-Rv2626c-RpfD
MDFALLPPEVNSARMYTGPGAGSLLAAAGGWDSLAAELATTAEAYGSVLSGLAALHWRGPAAESMAVTAAPYIGWLYTTAEKTQQTAIQARAAALAFEQAYAMTLPPPVVAANRIQLLALIATNFFGQNTAAIAATEAQYAEMWAQDAAAMYGYATASAAAALLTPFSPPRQTTNPAGLTAQAAAVSQATDPLSLLIETVTQALQALTIPSFIPEDFTFLDAIFAGYATVGVTQDVESFVAGTIGAESNLGLLNVGDENPAEVTPGDFGIGELVSATSPGGGVSASGAGGAASVGNTVLASVGRANSIGQLSVPPSWAAPSTRPVSALSPAGLTTLPGTDVAEHGMPGVPGVPVAAGRASGVLPRYGVRLTVMAHPPAAGEFMIATTRDREGATMITFRLRLPCRTILRVFSRNPLVRGTDRLEAVVMLLAVTVSLLTIPFAAAAGTAVQDSRSHVYAHQAQTRHPATATVIDHEGVIDSNTTATSAPPRTKITVPARWVVNGIERSGEVNAKPGTKSGDRVGIWVDSAGQLVDEPAPPARAIADAALAALGLWLSVAAVAGALLALTRAILIRVRNASWQHDIDSLFCTQRELMTTARDIMNAGVTCVGEHETLTAAAQYMREHDIGALPICGDDDRLHGMLTDRDIVIKGLAAGLDPNTATAGELARDSIYYVDANASIQEMLNVMEEHQVRRVPVISEHRLVGIVTEADIARHLPEHAIVQFVKAICSPMALASRQKGDTKFILNAKLLLGLSTISSKADDIDWDAIAQCESGGNWAANTGNGLYGGLQISQATWDSNGGVGSPAAASPQQQIEVADNIMKTQGPGAWPKCSSCSQGDAPLGSLTHILTFLAAETGGCSGSRDDKMK

SEQ ID NO: 73 - DNA, 3567 bp, synthetic construct
  source 1..3567: mol_type = other DNA
  misc_feature 1..3567: note = Description of Artificial Sequence: Mycobacterium PPE51-Rv1733c-Rv2626c-RpfB fusion protein
atggattttgcgctgctgccgccggaagtgaacagcgcgcgcatgtataccggcccgggcgcgggcagcctgctggcggcggcgggcggctgggatagcctggcggcggaactggcgaccaccgcggaagcgtatggcagcgtgctgagcggcctggcggcgctgcattggcgcggcccggcggcggaaagcatggcggtgaccgcggcgccgtatattggctggctgtataccaccgcggaaaaaacccagcagaccgcgattcaggcgcgcgcggcggcgctggcgtttgaacaggcgtatgcgatgaccctgccgccgccggtggtggcggcgaaccgcattcagctgctggcgctgattgcgaccaacttttttggccagaacaccgcggcgattgcggcgaccgaagcgcagtatgcggaaatgtgggcgcaggatgcggcggcgatgtatggctatgcgaccgcgagcgcggcggcggcgctgctgaccccgtttagcccgccgcgccagaccaccaacccggcgggcctgaccgcgcaggcggcggcggtgagccaggcgaccgatccgctgagcctgctgattgaaaccgtgacccaggcgctgcaggcgctgaccattccgagctttattccggaagattttacctttctggatgcgatttttgcgggctatgcgaccgtgggcgtgacccaggatgtggaaagctttgtggcgggcaccattggcgcggaaagcaacctgggcctgctgaacgtgggcgatgaaaacccggcggaagtgaccccgggcgattttggcattggcgaactggtgagcgcgaccagcccgggcggcggcgtgagcgcgagcggcgcgggcggcgcggcgagcgtgggcaacaccgtgctggcgagcgtgggccgcgcgaacagcattggccagctgagcgtgccgccgagctgggcggcgccgagcacccgcccggtgagcgcgctgagcccggcgggcctgaccaccctgccgggcaccgatgtggcggaacatggcatgccgggcgtgccgggcgtgccggtggcggcgggccgcgcgagcggcgtgctgccgcgctatggcgtgcgcctgaccgtgatggcgcatccgccggcggcgggcgaatttatgacagagcagcagtggaatttcgcgggtatcgaggccgcggcaagcgcaatccagggaaatgtcacgtccattcattccctccttgacgaggggaagcagtccctgaccaagctcgcagcggcctggggcggtagcggttcggaggcgtaccagggtgtccagcaaaaatgggacgccacggctaccgagctgaacaacgcgctgcagaacctggcgcggacgatcagcgaagccggtcaggcaatggcttcgaccgaaggcaacgtcactgggatgttcgcagaattcatgattgcgactacccgtgatcgtgagggcgcgaccatgatcacgttccgtctgcgtctgccgtgtcgcaccattttgcgcgtgttttcgcgtaacccgctggtccgcggtaccgaccgtctggaggccgttgtcatgctgctggcggttaccgtgagcctgctgacgatcccattcgcagcggcagctggcacggccgtccaagacagccgtagccatgtgtatgctcaccaggctcaaacccgtcacccggctactgccactgttatcgatcacgaaggcgtgattgactccaataccacggcaacctccgcaccgcctcgcaccaagattacggttcctgcgcgttgggtggtgaatggtattgaacgcagcggcgaagttaatgccaaaccgggtaccaaaagcggtgaccgtgtgggcatctgggtcgatagcgccggtcagctggtcgacgagccggcaccgccagcgcgtgcgatcgccgatgcggcgctggctgccctgggtctgtggctgagcgtggcagcggtcgccggtgcgttgctggcgctgacgcgcgcaattctgatccgcgttcgcaatgcgagctggcagcacgatattgatagcctgttttgcacccaacgtgagctcatgaccacggcgcgtgatatcatgaatgcgggtgtcacctgtgttggcgagcacgaaacgttgaccgcagcagcacagtacatgcgcgaacatgatatcggcgcattgccgatttgcggcgacgatgatcgtctgcacggtatgctgaccgaccgcgatatcgttatcaagggtctggccgcaggcttggacccgaacaccgcgaccgccggtgaactggcacgtgacagcatctattacgtcgacgcgaacgccagcattcaagagatgctgaacgtgatggaagagcatcaggtgcgtcgtgtcccggttatcagcgaacatcgtctggttggtatcgttaccgaagccgacatcgcacgtcacctgccggagcacgcgattgttcagttcgtgaaagcgatttgcagcccgatggcgttggcgtctcgtcaaaagggcgacacaaaatttattctaaatgcaaagcttgcatgcaaaacggtgacgttgaccgtcgacggaaccgcgatgcgggtgaccacgatgaaatcgcgggtgatcgacatcgtcgaagagaacgggttctcagtcgacgaccgcgacgacctgtatcccgcggccggcgtgcaggtccatgacgccgacaccatcgtgctgcggcgtagccgtccgctgcagatctcgctggatggtcacgacgctaagcaggtgtggacgaccgcgtcgacggtggacgaggcgctggcccaactcgcgatgaccgacacggcgccggccgcggcttctcgcgccagccgcgtcccgctgtccgggatggcgctaccggtcgtcagcgccaagacggtgcagctcaacgacggcgggttggtgcgcacggtgcacttgccggcccccaatgtcgcggggctgctgagtgcggccggcgtgccgctgttgcaaagcgaccacgtggtgcccgccgcgacggccccgatcgtcgaaggcatgcagatccaggtgacccgcaatcggatcaagaaggtcaccgagcggctgccgctgccgccgaacgcgcgtcgtgtcgaggacccggagatgaacatgagccgggaggtcgtcgaagacccgggggttccggggacccaggatgtgacgttcgcggtagctgaggtcaacggcgtcgagaccggccgtttgcccgtcgccaacgtcgtggtgaccccggcccacgaagccgtggtgcgggtgggcaccaagcccggtaccgaggtgcccccggtgatcgacggaagcatctgggacgcgatcgccggctgtgaggccggtggcaactgggcgatcaacaccggcaacgggtattacggtggtgtgcagtttgaccagggcacctgggaggccaacggcgggctgcggtatgcaccccgcgctgacctcgccacccgcgaagagcagatcgccgttgccgaggtgacccgactgcgtcaaggttggggcgcctggccggtatgtgctgcacgagcgggtgcgcgctga

SEQ ID NO: 74 - protein, 1091 aa, synthetic construct
  SOURCE 1..1091
  REGION 1..1091: NOTE = Description of Artificial Sequence: PPE51-Rv1733c-Rv2626c-RpfB
MDFALLPPEVNSARMYTGPGAGSLLAAAGGWDSLAAELATTAEAYGSVLSGLAALHWRGPAAESMAVTAAPYIGWLYTTAEKTQQTAIQARAAALAFEQAYAMTLPPPVVAANRIQLLALIATNFFGQNTAAIAATEAQYAEMWAQDAAAMYGYATASAAAALLTPFSPPRQTTNPAGLTAQAAAVSQATDPLSLLIETVTQALQALTIPSFIPEDFTFLDAIFAGYATVGVTQDVESFVAGTIGAESNLGLLNVGDENPAEVTPGDFGIGELVSATSPGGGVSASGAGGAASVGNTVLASVGRANSIGQLSVPPSWAAPSTRPVSALSPAGLTTLPGTDVAEHGMPGVPGVPVAAGRASGVLPRYGVRLTVMAHPPAAGEFMIATTRDREGATMITFRLRLPCRTILRVFSRNPLVRGTDRLEAVVMLLAVTVSLLTIPFAAAAGTAVQDSRSHVYAHQAQTRHPATATVIDHEGVIDSNTTATSAPPRTKITVPARWVVNGIERSGEVNAKPGTKSGDRVGIWVDSAGQLVDEPAPPARAIADAALAALGLWLSVAAVAGALLALTRAILIRVRNASWQHDIDSLFCTQRELMTTARDIMNAGVTCVGEHETLTAAAQYMREHDIGALPICGDDDRLHGMLTDRDIVIKGLAAGLDPNTATAGELARDSIYYVDANASIQEMLNVMEEHQVRRVPVISEHRLVGIVTEADIARHLPEHAIVQFVKAICSPMALASRQKGDTKFILNAKLACKTVTLTVDGTAMRVTTMKSRVIDIVEENGFSVDDRDDLYPAAGVQVHDADTIVLRRSRPLQISLDGHDAKQVWTTASTVDEALAQLAMTDTAPAAASRASRVPLSGMALPVVSAKTVQLNDGGLVRTVHLPAPNVAGLLSAAGVPLLQSDHVVPAATAPIVEGMQIQVTRNRIKKVTERLPLPPNARRVEDPEMNMSREVVEDPGVPGTQDVTFAVAEVNGVETGRLPVANVVVTPAHEAVVRVGTKPGTEVPPVIDGSIWDAIAGCEAGGNWAINTGNGYYGGVQFDQGTWEANGGLRYAPRADLATREEQIAVAEVTRLRQGWGAWPVCAARAGAR

SEQ ID NO: 75 - DNA, 31 bp, synthetic construct
  source 1..31: mol_type = other DNA
  misc_feature 1..31: note = Description of Artificial Sequence: 85B For NdeI primer
atagatcatatgtttagccgtcctggcctgc

SEQ ID NO: 76 - DNA, 31 bp, synthetic construct
  source 1..31: mol_type = other DNA
  misc_feature 1..31: note = Description of Artificial Sequence: 85B Rev EcoRI nostop primer
ttaagagaattcgcccgcacccagagaggat

SEQ ID NO: 77 - DNA, 32 bp, synthetic construct
  source 1..32: mol_type = other DNA
  misc_feature 1..32: note = Description of Artificial Sequence: ESAT-6 For BamHI primer
aacgttggatccatgacagagcagcagtggaa

SEQ ID NO: 78 - DNA, 32 bp, synthetic construct
  source 1..32: mol_type = other DNA
  misc_feature 1..32: note = Description of Artificial Sequence: ESAT-6 Rev EcoRI ns primer
atactagaattctgcgaacatcccagtgacgt

SEQ ID NO: 79 - DNA, 33 bp, synthetic construct
  source 1..33: mol_type = other DNA
  misc_feature 1..33: note = Description of Artificial Sequence: 1733 For EcoRI primer
aacttagaattcatgattgcgactacccgtgat

SEQ ID NO: 80 - DNA, 30 bp, synthetic construct
  source 1..30: mol_type = other DNA
  misc_feature 1..30: note = Description of Artificial Sequence: 1733 In1 Rev Xma primer
gatatacccgggggcctccagacggtcggt

SEQ ID NO: 81 - DNA, 31 bp, synthetic construct
  source 1..31: mol_type = other DNA
  misc_feature 1..31: note = Description of Artificial Sequence: 1733 Out For Xma primer
aacgaacccggggtccaagacagccgtagcc

SEQ ID NO: 82 - DNA, 31 bp, synthetic construct
  source 1..31: mol_type = other DNA
  misc_feature 1..31: note = Description of Artificial Sequence: 1733 Out Rev Xba primer
taagtatctagaatcggcgatcgcacgcgct

SEQ ID NO: 83 - DNA, 32 bp, synthetic construct
  source 1..32: mol_type = other DNA
  misc_feature 1..32: note = Description of Artificial Sequence: 1733 In2 For Xba primer
atagaatctagacgcgcaattctgatccgcgt

SEQ ID NO: 84 - DNA, 32 bp, synthetic construct
  source 1..32: mol_type = other DNA
  misc_feature 1..32: note = Description of Artificial Sequence: 1733 Rev ns SacI primer
agataagagctcacgttgggtgcaaaacaggc

SEQ ID NO: 85 - DNA, 31 bp, synthetic construct
  source 1..31: mol_type = other DNA
  misc_feature 1..31: note = Description of Artificial Sequence: 2626 For SacI primer
atagaagagctcatgaccacggcgcgtgata

SEQ ID NO: 86 - DNA, 36 bp, synthetic construct
  source 1..36: mol_type = other DNA
  misc_feature 1..36: note = Description of Artificial Sequence: 2626 Rev HindIII ns primer
taaagaaagctttgcatttagaataaattttgtgtc

SEQ ID NO: 87 - DNA, 30 bp, synthetic construct
  source 1..30: mol_type = other DNA
  misc_feature 1..30: note = Description of Artificial Sequence: RpfD For HindIII primer
taactaaagcttttgctgggcctgagcacc

SEQ ID NO: 88 - DNA, 33 bp, synthetic construct
  source 1..33: mol_type = other DNA
  misc_feature 1..33: note = Description of Artificial Sequence: RpfD Rev XhoI stop primer
atctaactcgagctagtcatcgcggctaccgct

SEQ ID NO: 89 - DNA, 33 bp, synthetic construct
  source 1..33: mol_type = other DNA
  misc_feature 1..33: note = Description of Artificial Sequence: ESAT6 For NdeI primer
taagatcatatgacagagcagcagtggaatttc

SEQ ID NO: 90 - DNA, 32 bp, synthetic construct; identical to SEQ ID NO: 78
  source 1..32: mol_type = other DNA
  misc_feature 1..32: note = Description of Artificial Sequence: ESAT-6 Rev EcoRI ns primer

SEQ ID NO: 91 - DNA, 1263 bp, synthetic construct
  source 1..1263: mol_type = other DNA
  misc_feature 1..1263: note = Description of Artificial Sequence: Ag85B-ESAT6 fusion protein withAg85B signal sequence
atgacagacgtgagccgaaagattcgagcttggggacgccgattgatgatcggcacggcagcggctgtagtccttccgggcctggtggggcttgccggcggagcggcaaccgcgggcgcgttctcccggccggggctgccggtcgagtacctgcaggtgccgtcgccgtcgatgggccgcgacatcaaggttcagttccagagcggtgggaacaactcacctgcggtttatctgctcgacggcctgcgcgcccaagacgactacaacggctgggatatcaacaccccggcgttcgagtggtactaccagtcgggactgtcgatagtcatgccggtcggcgggcagtccagcttctacagcgactggtacagcccggcctgcggtaaggctggctgccagacttacaagtgggaaaccttcctgaccagcgagctgccgcaatggttgtccgccaacagggccgtgaagcccaccggcagcgctgcaatcggcttgtcgatggccggctcgtcggcaatgatcttggccgcctaccacccccagcagttcatctacgccggctcgctgtcggccctgctggacccctctcaggggatggggcctagcctgatcggcctcgcgatgggtgacgccggcggttacaaggccgcagacatgtggggtccctcgagtgacccggcatgggagcgcaacgaccctacgcagcagatccccaagctggtcgcaaacaacacccggctatgggtttattgcgggaacggcaccccgaacgagttgggcggtgccaacatacccgccgagttcttggagaacttcgttcgtagcagcaacctgaagttccaggatgcgtacaacgccgcgggcgggcacaacgccgtgttcaacttcccgcccaacggcacgcacagctgggagtactggggcgctcagctcaacgccatgaagggtgacctgcagagttcgttaggcgccggcatgacagagcagcagtggaatttcgcgggtatcgaggccgcggcaagcgcaatccagggaaatgtcacgtccattcattccctccttgacgaggggaagcagtccctgaccaagctcgcagcggcctggggcggtagcggttcggaggcgtaccagggtgtccagcaaaaatgggacgccacggctaccgagctgaacaacgcgctgcagaacctggcgcggacgatcagcgaagccggtcaggcaatggcttcgaccgaaggcaacgtcactgggatgttcgcatga

SEQ ID NO: 92 - protein, 420 aa, synthetic construct
  SOURCE 1..420
  REGION 1..420: NOTE = Description of Artificial Sequence: Ag85B-ESAT6 (Ag85B signalsequence)
MTDVSRKIRAWGRRLMIGTAAAVVLPGLVGLAGGAATAGAFSRPGLPVEYLQVPSPSMGRDIKVQFQSGGNNSPAVYLLDGLRAQDDYNGWDINTPAFEWYYQSGLSIVMPVGGQSSFYSDWYSPACGKAGCQTYKWETFLTSELPQWLSANRAVKPTGSAAIGLSMAGSSAMILAAYHPQQFIYAGSLSALLDPSQGMGPSLIGLAMGDAGGYKAADMWGPSSDPAWERNDPTQQIPKLVANNTRLWVYCGNGTPNELGGANIPAEFLENFVRSSNLKFQDAYNAAGGHNAVFNFPPNGTHSWEYWGAQLNAMKGDLQSSLGAGMTEQQWNFAGIEAAASAIQGNVTSIHSLLDEGKQSLTKLAAAWGGSGSEAYQGVQQKWDATATELNNALQNLARTISEAGQAMASTEGNVTGMFA

SEQ ID NO: 93 - DNA, 1272 bp, synthetic construct
  source 1..1272: mol_type = other DNA
  misc_feature 1..1272: note = Description of Artificial Sequence: Ag85B-ESAT6 fusion protein with19 kDa lipoprotein signal sequence
atgaagcgtggactgacggtcgcggtagccggagccgccattctggtcgcaggtctttccggatgttcaagcaacaagtcgactacaggaagcggtgagaccacgaccgcggcaggtaccacggcaagccccggccggccggggctgccggtcgagtacctgcaggtgccgtcgccgtcgatgggccgcgacatcaaggttcagttccagagcggtgggaacaactcacctgcggtttatctgctcgacggcctgcgcgcccaagacgactacaacggctgggatatcaacaccccggcgttcgagtggtactaccagtcgggactgtcgatagtcatgccggtcggcgggcagtccagcttctacagcgactggtacagcccggcctgcggtaaggctggctgccagacttacaagtgggaaaccttcctgaccagcgagctgccgcaatggttgtccgccaacagggccgtgaagcccaccggcagcgctgcaatcggcttgtcgatggccggctcgtcggcaatgatcttggccgcctaccacccccagcagttcatctacgccggctcgctgtcggccctgctggacccctctcaggggatggggcctagcctgatcggcctcgcgatgggtgacgccggcggttacaaggccgcagacatgtggggtccctcgagtgacccggcatgggagcgcaacgaccctacgcagcagatccccaagctggtcgcaaacaacacccggctatgggtttattgcgggaacggcaccccgaacgagttgggcggtgccaacatacccgccgagttcttggagaacttcgttcgtagcagcaacctgaagttccaggatgcgtacaacgccgcgggcgggcacaacgccgtgttcaacttcccgcccaacggcacgcacagctgggagtactggggcgctcagctcaacgccatgaagggtgacctgcagagttcgttaggcgccggcatgacagagcagcagtggaatttcgcgggtatcgaggccgcggcaagcgcaatccagggaaatgtcacgtccattcattccctccttgacgaggggaagcagtccctgaccaagctcgcagcggcctggggcggtagcggttcggaggcgtaccagggtgtccagcaaaaatgggacgccacggctaccgagctgaacaacgcgctgcagaacctggcgcggacgatcagcgaagccggtcaggcaatggcttcgaccgaaggcaacgtcactgggatgttcgcatga

SEQ ID NO: 94 - protein, 423 aa, synthetic construct
  SOURCE 1..423
  REGION 1..423: NOTE = Description of Artificial Sequence: Ag85B-ESAT6 (19 kDa lipoproteinsignal sequence)
MKRGLTVAVAGAAILVAGLSGCSSNKSTTGSGETTTAAGTTASPGRPGLPVEYLQVPSPSMGRDIKVQFQSGGNNSPAVYLLDGLRAQDDYNGWDINTPAFEWYYQSGLSIVMPVGGQSSFYSDWYSPACGKAGCQTYKWETFLTSELPQWLSANRAVKPTGSAAIGLSMAGSSAMILAAYHPQQFIYAGSLSALLDPSQGMGPSLIGLAMGDAGGYKAADMWGPSSDPAWERNDPTQQIPKLVANNTRLWVYCGNGTPNELGGANIPAEFLENFVRSSNLKFQDAYNAAGGHNAVFNFPPNGTHSWEYWGAQLNAMKGDLQSSLGAGMTEQQWNFAGIEAAASAIQGNVTSIHSLLDEGKQSLTKLAAAWGGSGSEAYQGVQQKWDATATELNNALQNLARTISEAGQAMASTEGNVTGMFA

SEQ ID NO: 95 - DNA, 1020 bp, synthetic construct
  source 1..1020: mol_type = other DNA
  misc_feature 1..1020: note = Description of Artificial Sequence: Rv2626c-RpfD fusion proteinwith Ag85B signal sequence
atgacagacgtgagccgaaagattcgagcttggggacgccgattgatgatcggcacggcagcggctgtagtccttccgggcctggtggggcttgccggcggagcggcaaccgcgggcgcgttctccatgaccaccgcacgcgacatcatgaacgcaggtgtgacctgtgttggcgaacacgagacgctaaccgctgccgctcaatacatgcgtgagcacgacatcggcgcgttgccgatctgcggggacgacgaccggctgcacggcatgctcaccgaccgcgacattgtgatcaaaggcctggctgcgggcctagacccgaataccgccacggctggcgagttggcccgggacagcatctactacgtcgatgcgaacgcaagcatccaggagatgctcaacgtcatggaagaacatcaggtccgccgtgttccggtcatctcagagcaccgcttggtcggaatcgtcaccgaagccgacatcgcccgacacctgcccgagcacgccattgtgcagttcgtcaaggcaatctgctcgcccatggccctcgccagcatgacaccgggtttgcttactactgcgggtgctggccgaccacgtgacaggtgcgccaggatcgtatgcacggtgttcatcgaaaccgccgttgtcgcgaccatgtttgtcgcgttgttgggtctgtccaccatcagctcgaaagccgacgacatcgattgggacgccatcgcgcaatgcgaatccggcggcaattgggcggccaacaccggtaacgggttatacggtggtctgcagatcagccaggcgacgtgggattccaacggtggtgtcgggtcgccggcggccgcgagtccccagcaacagatcgaggtcgcagacaacattatgaaaacccaaggcccgggtgcgtggccgaaatgtagttcttgtagtcagggagacgcaccgctgggctcgctcacccacatcctgacgttcctcgcggccgagactggaggttgttcggggagcagggacgattag

SEQ ID NO: 96 - protein, 339 aa, synthetic construct
  SOURCE 1..339
  REGION 1..339: NOTE = Description of Artificial Sequence: Rv2626c-RpfD (Ag85B signalsequence)
MTDVSRKIRAWGRRLMIGTAAAVVLPGLVGLAGGAATAGAFSMTTARDIMNAGVTCVGEHETLTAAAQYMREHDIGALPICGDDDRLHGMLTDRDIVIKGLAAGLDPNTATAGELARDSIYYVDANASIQEMLNVMEEHQVRRVPVISEHRLVGIVTEADIARHLPEHAIVQFVKAICSPMALASMTPGLLTTAGAGRPRDRCARIVCTVFIETAVVATMFVALLGLSTISSKADDIDWDAIAQCESGGNWAANTGNGLYGGLQISQATWDSNGGVGSPAAASPQQQIEVADNIMKTQGPGAWPKCSSCSQGDAPLGSLTHILTFLAAETGGCSGSRDD

SEQ ID NO: 97 - DNA, 1029 bp, synthetic construct
  source 1..1029: mol_type = other DNA
  misc_feature 1..1029: note = Description of Artificial Sequence: Rv2626c-RpfD fusion proteinwith 19 kDa lipoprotein signal sequence
atgaagcgtggactgacggtcgcggtagccggagccgccattctggtcgcaggtctttccggatgttcaagcaacaagtcgactacaggaagcggtgagaccacgaccgcggcaggtaccacggcaagccccggcatgaccaccgcacgcgacatcatgaacgcaggtgtgacctgtgttggcgaacacgagacgctaaccgctgccgctcaatacatgcgtgagcacgacatcggcgcgttgccgatctgcggggacgacgaccggctgcacggcatgctcaccgaccgcgacattgtgatcaaaggcctggctgcgggcctagacccgaataccgccacggctggcgagttggcccgggacagcatctactacgtcgatgcgaacgcaagcatccaggagatgctcaacgtcatggaagaacatcaggtccgccgtgttccggtcatctcagagcaccgcttggtcggaatcgtcaccgaagccgacatcgcccgacacctgcccgagcacgccattgtgcagttcgtcaaggcaatctgctcgcccatggccctcgccagcatgacaccgggtttgcttactactgcgggtgctggccgaccacgtgacaggtgcgccaggatcgtatgcacggtgttcatcgaaaccgccgttgtcgcgaccatgtttgtcgcgttgttgggtctgtccaccatcagctcgaaagccgacgacatcgattgggacgccatcgcgcaatgcgaatccggcggcaattgggcggccaacaccggtaacgggttatacggtggtctgcagatcagccaggcgacgtgggattccaacggtggtgtcgggtcgccggcggccgcgagtccccagcaacagatcgaggtcgcagacaacattatgaaaacccaaggcccgggtgcgtggccgaaatgtagttcttgtagtcagggagacgcaccgctgggctcgctcacccacatcctgacgttcctcgcggccgagactggaggttgttcggggagcagggacgattag

SEQ ID NO: 98 - protein, 342 aa, synthetic construct
  REGION 1..342: NOTE = Description of Artificial Sequence: Rv2626c-RpfD (19 kDalipoprotein signal sequence)
  SOURCE 1..342
MKRGLTVAVAGAAILVAGLSGCSSNKSTTGSGETTTAAGTTASPGMTTARDIMNAGVTCVGEHETLTAAAQYMREHDIGALPICGDDDRLHGMLTDRDIVIKGLAAGLDPNTATAGELARDSIYYVDANASIQEMLNVMEEHQVRRVPVISEHRLVGIVTEADIARHLPEHAIVQFVKAICSPMALASMTPGLLTTAGAGRPRDRCARIVCTVFIETAVVATMFVALLGLSTISSKADDIDWDAIAQCESGGNWAANTGNGLYGGLQISQATWDSNGGVGSPAAASPQQQIEVADNIMKTQGPGAWPKCSSCSQGDAPLGSLTHILTFLAAETGGCSGSRDD